European Patent Specification EP 3 959 232 B1, published October 16, 2024. Title: AAV CAPSID CHIMERIC ANTIGEN RECEPTORS AND USES THEREOF. Applicant: University of Massachusetts. Application Not Yet Assigned. The sequence listing filed with the application follows.

SEQUENCE LISTING (39 sequences)

SEQ ID NO: 1 - DNA, 11147 bp, Unknown
  AAV-CAR-FoxP3-EGFRt
ctgttttaaaagaaaaggggggattggggggtacagtgcaggggaaagaatagtagacataatagcaacagacatacaaactaaagaattacaaaaacaaattacaaaaattcaaaattttatcaacaagcttgatcgatggctccggtgcccgtcagtgggcagagcgcacatcgcccacagtccccgagaagttggggggaggggtcggcaattgaaccggtgcctagagaaggtggcgcggggtaaactgggaaagtgatgtcgtgtactggctccgcctttttcccgagggtgggggagaaccgtatataagtgcagtagtcgccgtgaacgttctttttcgcaacgggtttgccgccagaacacaggtgtcgtgacgcggatccacgcgtgcggccgcacgcgtaagcttagcgcagaggcttggggcagccgagcggcagccaggccccggcccgggcctcggttccagaagggagaggagcccgccaaggcgcgcaagagagcgggctgcctcgcagtccgagccggagagggagcgcgagccgcgccggccccggacggcctcgccgccaccatggctctgcccgtcaccgcactgctgctgcctctggctctgctgctgcacgccgcaagaccagacattgtgctgacacagtctcctgcttccttagctgtatctctggggcagagggccaccatctcatgcagggccagccaaagtgtcagttcatctacctataattttatacactggtatcaacagaaatcaggacagccacccaaactcctcatcaagtatgcatccaacctagaatctggggtccctgtcaggttcagtggcagtgggtctgggacagacttctccctcaacatccatcctgtggaggaggaggatactgcaacatattactgtcagcacagttgggagattccatacacgttcggagggggggccaagttggagataaaaggcagtactagcggtggtggctccgggggcggttccggtgggggcggcagcagccaggtgcagctgaaggagtcaggacctggcctggtggcaccctcacagagcctgtccatcacatgcaccgtctcaggattctcattaagcggctatggcataagctgggttcgccagcctccaggaaagcgtctggaatggctgggattgatatggggtgatggaaccacagactataattcagctctcaaatccagactgagcatcagcaaggacaactccaagagccaggttttcttaaaaatgaacagtctgcaaactgatgacacagccaggtacttctgtaccagagggcctccggccttctataagtacctctactttgactactggggccaaggcaccactctcacagtctcctcagacaaaactcacacatgcccaccgtgcccagcacctcctgtggcaggaccgtcagtcttcctcttccccccaaaacccaaggacaccctcatgatctcccggacccctgaggtcacatgcgtggtggtggacgtgagccacgaagaccctgaggtcaagttcaactggtacgtggacggcgtggaggtgcataatgccaagacaaagccgcgggaggagcagtaccagagcacgtaccgtgtggtcagcgtcctcaccgtcctgcaccaggactggctgaatggcaaggagtacaagtgcaaggtctccaacaaagccctcccagcccccatcgagaaaaccatctccaaagccaaagggcagccccgagaaccacaggtgtacaccctgccaccatcacgagatgagctgaccaagaaccaggtcagcctgacctgcctggtcaaaggcttctatcccagcgacatcgccgtggagtgggagagcaatgggcagccggagaacaactacaagaccacgcctcccgtgctggactccgacggctccttcttcctctacagcaagctcaccgtggacaagagcaggtggcagcaggggaacgtcttctcatgctccgtgatgcatgaggctctgcacaaccactacacgcagaagagcctctccctgtctcccttttgggtgctggtggtggttggtggagtcctggcttgctatagcttgctagtaacagtggcctttattattttctgggtgaggagtaagaggagcaggggaggtcacagtgactacatgaacatgactccccgccgccccgggcccacccgcaagcattaccagccctatgccccaccacgcgacttcgcagcctatcgctccaaacggggcagaaagaaactcctgtatatattcaaacaaccatttatgagaccagtacaaactactcaagaggaagatggctgtagctgccgatttccagaagaagaagaaggaggatgtgaactgagagtgaagttcagcaggagcgcagacgcccccgcgtaccagcagggccagaaccagctctataacgagctcaatctaggacgaagagaggagtacgatgttttggacaagagacgtggccgggaccctgagatggggggaaagccgagaaggaagaaccctcaggaaggcctgtacaatgaactgcagaaagataagatggcggaggcctacagtgagattgggatgaaaggcgagcgccggaggggcaaggggcacgatggcctttaccagggtctcagtacagccaccaaggacacctacgacgcccttcacatgcaggccctgccccctcgccagtgtactaattatgctctcttgaaattggctggagatgttgagagcaaccccgggccggaattcatgcccaaccctaggccagccaagcctatggctccttccttggcccttggcccatccccaggagtcttgccaagctggaagactgcacccaagggctcagaacttctagggaccaggggctctgggggacccttccaaggtcgggacctgcgaagtggggcccacacctcttcttccttgaaccccctgccaccatcccagctgcagctgcctacagtgcccctagtcatggtggcaccgtctggggcccgactaggtccctcaccccacctacaggcccttctccaggacagaccacacttcatgcatcagctctccactgtggatgcccatgcccagacccctgtgctccaagtgcgtccactggacaacccagccatgatcagcctcccaccaccttctgctgccactggggtcttctccctcaaggcccggcctggcctgccacctgggatcaatgtggccagtctggaatgggtgtccagggagccagctctactctgcaccttcccacgctcgggtacacccaggaaagacagcaaccttttggctgcaccccaaggatcctacccactgctggcaaatggagtctgcaagtggcctggttgtgagaaggtcttcgaggagccagaagagtttctcaagcactgccaagcagatcatctcctggatgagaaaggcaaggcccagtgcctcctccagagagaagtggtgcagtctctggagcagcagctggagctggaaaaggagaagctgggagctatgcaggcccacctggctgggaagatggcgctggccaaggctccatctgtggcctcaatggacaagagctcttgctgcatcgtagccaccagtactcagggcagtgtgctcccggcctggtctgctcctcgggaggctccagacggcggcctgtttgcagtgcggaggcacctctggggaagccatggcaatagttccttcccagagttcttccacaacatggactacttcaagtaccacaatatgcgaccccctttcacctatgccacccttatccgatgggccatcctggaagccccggagaggcagaggacactcaatgaaatctaccattggtttactcgcatgttcgcctacttcagaaaccaccccgccacctggaagaatgccatccgccacaacctgagcctgcacaagtgctttgtgcgagtggagagcgagaagggagcagtgtggaccgtagatgaatttgagtttcgcaagaagaggagccaacgccccaacaagtgctccaatccctgccctgaattctctagacagtgtactaattatgctctcttgaaattggctggagatgttgagagcaaccccgggccgatgcttctcctggtgacaagccttctgctctgtgagttaccacacccagcattcctcctgatcccacgcaaagtgtgtaacggaataggtattggtgaatttaaagactcactctccataaatgctacgaatattaaacacttcaaaaactgcacctccatcagtggcgatctccacatcctgccggtggcatttaggggtgactccttcacacatactcctcctctggatccacaggaactggatattctgaaaaccgtaaaggaaatcacagggtttttgctgattcaggcttggcctgaaaacaggacggacctccatgcctttgagaacctagaaatcatacgcggcaggaccaagcaacatggtcagttttctcttgcagtcgtcagcctgaacataacatccttgggattacgctccctcaaggagataagtgatggagatgtgataatttcaggaaacaaaaatttgtgctatgcaaatacaataaactggaaaaaactgtttgggacctccggtcagaaaaccaaaattataagcaacagaggtgaaaacagctgcaaggccacaggccaggtctgccatgccttgtgctcccccgagggctgctggggcccggagcccagggactgcgtctcttgccggaatgtcagccgaggcagggaatgcgtggacaagtgcaaccttctggagggtgagccaagggagtttgtggagaactctgagtgcatacagtgccacccagagtgcctgcctcaggccatgaacatcacctgcacaggacggggaccagacaactgtatccagtgtgcccactacattgacggcccccactgcgtcaagacctgcccggcaggagtcatgggagaaaacaacaccctggtctggaagtacgcagacgccggccatgtgtgccacctgtgccatccaaactgcacctacggatgcactgggccaggtcttgaaggctgtccaacgaatgggcctaagatcccgtccatcgccactggatctagataaattcgagcatcttaccgccatttattcccatatttgttctgtttttcttgatttgggtatacatttaaatgttaataaaacaaaatggtggggcaatcatttacatttttagggatatgtaattactagttcaggtgtattgccacaagacaaacatgttaagaaactttcccgttatttacgctctgttcctgttaatcaacctctggattacaaaatttgtgaaagattgactgatattcttaactatgttgctccttttacgctgtgtggatatgctgctttatagcctctgtatctagctattgcttcccgtacggctttcgttttctcctccttgtataaatcctggttgctgtctcttttagaggagttgtggcccgttgtccgtcaacgtggcgtggtgtgctctgtgtttgctgacgcaacccccactggctggggcattgccaccacctgtcaactcctttctgggactttcgctttccccctcccgatcgccacggcagaactcatcgccgcctgccttgcccgctgctggacaggggctaggttgctgggcactgataattccgtggtgttgtcggggaagctgacgtcctttcctcgagggggggcccggtacctttaagaccaatgacttacaaggcagctgtagatcttagccactttttaaaagaaaaggggggactggaagggctaattcactcccaacgaagacaagatctgctttttgcttgtactgggtctctctggttagaccagatctgagcctgggagctctctggctaactagggaacccactgcttaagcctcaataaagcttgccttgagtgcttcaagtagtgtgtgcccgtctgttgtgtgactctggtaactagagatccctcagacccttttagtcagtgtggaaaatctctagcagtagtagttcatgtcatcttattattcagtatttataacttgcaaagaaatgaatatcagagagtgagaggaacttgtttattgcagcttataatggttacaaataaagcaatagcatcacaaatttcacaaataaagcatttttttcactgcattctagttgtggtttgtccaaactcatcaatgtatcttatcatgtctggctctagctatcccgcccctaactccgcccagttccgcccattctccgccccatggctgactaattttttttatttatgcagaggccgaggccgcctcggcctctgagctattccagaagtagtgaggaggcttttttggaggcctaggcttttgcgtcgagacgtacccaattcgccctatagtgagtcgtattacgcgcgctcactggccgtcgttttacaacgtcgtgactgggaaaaccctggcgttacccaacttaatcgccttgcagcacatccccctttcgccagctggcgtaatagcgaagaggcccgcaccgatcgcccttcccaacagttgcgcagcctgaatggcgaatggcgcgacgcgccctgtagcggcgcattaagcgcggcgggtgtggtggttacgcgcagcgtgaccgctacacttgccagcgccctagcgcccgctcctttcgctttcttcccttcctttctcgccacgttcgccggctttccccgtcaagctctaaatcgggggctccctttagggttccgatttagtgctttacggcacctcgaccccaaaaaacttgattagggtgatggttcacgtagtgggccatcgccctgatagacggtttttcgccctttgacgttggagtccacgttctttaatagtggactcttgttccaaactggaacaacactcaaccctatctcggtctattcttttgatttataagggattttgccgatttcggcctattggttaaaaaatgagctgatttaacaaaaatttaacgcgaattttaacaaaatattaacgtttacaatttcccaggtggcacttttcggggaaatgtgcgcggaacccctatttgtttatttttctaaatacattcaaatatgtatccgctcatgagacaataaccctgataaatgcttcaataatattgaaaaaggaagagtatgagtattcaacatttccgtgtcgcccttattcccttttttgcggcattttgccttcctgtttttgctcacccagaaacgctggtgaaagtaaaagatgctgaagatcagttgggtgcacgagtgggttacatcgaactggatctcaacagcggtaagatccttgagagttttcgccccgaagaacgttttccaatgatgagcacttttaaagttctgctatgtggcgcggtattatcccgtattgacgccgggcaagagcaactcggtcgccgcatacactattctcagaatgacttggttgagtactcaccagtcacagaaaagcatcttacggatggcatgacagtaagagaattatgcagtgctgccataaccatgagtgataacactgcggccaacttacttctgacaacgatcggaggaccgaaggagctaaccgcttttttgcacaacatgggggatcatgtaactcgccttgatcgttgggaaccggagctgaatgaagccataccaaacgacgagcgtgacaccacgatgcctgtagcaatggcaacaacgttgcgcaaactattaactggcgaactacttactctagcttcccggcaacaattaatagactggatggaggcggataaagttgcaggaccacttctgcgctcggcccttccggctggctggtttattgctgataaatctggagccggtgagcgtgggtctcgcggtatcattgcagcactggggccagatggtaagccctcccgtatcgtagttatctacacgacggggagtcaggcaactatggatgaacgaaatagacagatcgctgagataggtgcctcactgattaagcattggtaactgtcagaccaagtttactcatatatactttagattgatttaaaacttcatttttaatttaaaaggatctaggtgaagatcctttttgataatctcatgaccaaaatcccttaacgtgagttttcgttccactgagcgtcagaccccgtagaaaagatcaaaggatcttcttgagatcctttttttctgcgcgtaatctgctgcttgcaaacaaaaaaaccaccgctaccagcggtggtttgtttgccggatcaagagctaccaactctttttccgaaggtaactggcttcagcagagcgcagataccaaatactgtccttctagtgtagccgtagttaggccaccacttcaagaactctgtagcaccgcctacatacctcgctctgctaatcctgttaccagtggctgctgccagtggcgataagtcgtgtcttaccgggttggactcaagacgatagttaccggataaggcgcagcggtcgggctgaacggggggttcgtgcacacagcccagcttggagcgaacgacctacaccgaactgagatacctacagcgtgagctatgagaaagcgccacgcttcccgaagggagaaaggcggacaggtatccggtaagcggcagggtcggaacaggagagcgcacgagggagcttccagggggaaacgcctggtatctttatagtcctgtcgggtttcgccacctctgacttgagcgtcgatttttgtgatgctcgtcaggggggcggagcctatggaaaaacgccagcaacgcggcctttttacggttcctggccttttgctggccttttgctcacatgttctttcctgcgttatcccctgattctgtggataaccgtattaccgcctttgagtgagctgataccgctcgccgcagccgaacgaccgagcgcagcgagtcagtgagcgaggaagcggaagagcgcccaatacgcaaaccgcctctccccgcgcgttggccgattcattaatgcagctggcacgacaggtttcccgactggaaagcgggcagtgagcgcaacgcaattaatgtgagttagctcactcattaggcaccccaggctttacactttatgcttccggctcgtatgttgtgtggaattgtgagcggataacaatttcacacaggaaacagctatgaccatgattacgccaagcgcgcaattaaccctcactaaagggaacaaaagctggagctgcaagcttaatgtagtcttatgcaatactcttgtagtcttgcaacatggtaacgatgagttagcaacatgccttacaaggagagaaaaagcaccgtgcatgccgattggtggaagtaaggtggtacgatcgtgccttattaggaaggcaacagacgggtctgacatggattggacgaaccactgaattgccgcattgcagagatattgtatttaagtgcctagctcgatacataaacgggtctctctggttagaccagatctgagcctgggagctctctggctaactagggaacccactgcttaagcctcaataaagcttgccttgagtgcttcaagtagtgtgtgcccgtctgttgtgtgactctggtaactagagatccctcagacccttttagtcagtgtggaaaatctctagcagtggcgcccgaacagggacttgaaagcgaaagggaaaccagaggagctctctcgacgcaggactcggcttgctgaagcgcgcacggcaagaggcgaggggcggcgactggtgagtacgccaaaaattttgactagcggaggctagaaggagagagatgggtgcgagagcgtcagtattaagcgggggagaattagatcgcgatgggaaaaaattcggttaaggccagggggaaagaaaaaatataaattaaaacatatagtatgggcaagcagggagctagaacgattcgcagttaatcctggcctgttagaaacatcagaaggctgtagacaaatactgggacagctacaaccatcccttcagacaggatcagaagaacttagatcattatataatacagtagcaaccctctattgtgtgcatcaaaggatagagataaaagacaccaaggaagctttagacaagatagaggaagagcaaaacaaaagtaagaccaccgcacagcaagcggccgctgatcttcagacctggaggaggagatatgagggacaattggagaagtgaattatataaatataaagtagtaaaaattgaaccattaggagtagcacccaccaaggcaaagagaagagtggtgcagagagaaaaaagagcagtgggaataggagctttgttccttgggttcttgggagcagcaggaagcactatgggcgcagcctcaatgacgctgacggtacaggccagacaattattgtctggtatagtgcagcagcagaacaatttgctgagggctattgaggcgcaacagcatctgttgcaactcacagtctggggcatcaagcagctccaggcaagaatcctggctgtggaaagatacctaaaggatcaacagctcctggggatttggggttgctctggaaaactcatttgcaccactgctgtgccttggaatgctagttggagtaataaatctctggaacagatttggaatcacacgacctggatggagtgggacagagaaattaacaattacacaagcttaatacactccttaattgaagaatcgcaaaaccagcaagaaaagaatgaacaagaattattggaattagataaatgggcaagtttgtggaattggtttaacataacaaattggctgtggtatataaaattattcataatgatagtaggaggcttggtaggtttaagaatagtttttgctgtactttctatagtgaatagagttaggcagggatattcaccattatcgtttcagacccacctcccaaccccgaggggacccgacaggcccgaaggaatagaagaagaaggtggagagagagacagagacagatccattcgattagtgaacggatctcgacggtatcggtt

SEQ ID NO: 2 - DNA, 10047 bp, Unknown
  14-2_Lenti-IF5-D3-NQ-28-BB-Z
ctgttttaaaagaaaaggggggattggggggtacagtgcaggggaaagaatagtagacataatagcaacagacatacaaactaaagaattacaaaaacaaattacaaaaattcaaaattttatcaacaagcttgatcgatggctccggtgcccgtcagtgggcagagcgcacatcgcccacagtccccgagaagttggggggaggggtcggcaattgaaccggtgcctagagaaggtggcgcggggtaaactgggaaagtgatgtcgtgtactggctccgcctttttcccgagggtgggggagaaccgtatataagtgcagtagtcgccgtgaacgttctttttcgcaacgggtttgccgccagaacacaggtgtcgtgacgcggatccacgcgtgcggccgcacgcgtaagcttagcgcagaggcttggggcagccgagcggcagccaggccccggcccgggcctcggttccagaagggagaggagcccgccaaggcgcgcaagagagcgggctgcctcgcagtccgagccggagagggagcgcgagccgcgccggccccggacggcctcgccgccaccatggagacagacacactcctgctatgggtgctgctgctctgggttccaggttccactggtgacattgtgctgacacagtctcctgcttccttagctgtatctctggggcagagggccaccatctcatgcagggccagccaaagtgtcagttcatctacctataattttatacactggtatcaacagaaatcaggacagccacccaaactcctcatcaagtatgcatccaacctagaatctggggtccctgtcaggttcagtggcagtgggtctgggacagacttctccctcaacatccatcctgtggaggaggaggatactgcaacatattactgtcagcacagttgggagattccatacacgttcggagggggggccaagttggagataaaaggcagtactagcggtggtggctccgggggcggttccggtgggggcggcagcagccaggtgcagctgaaggagtcaggacctggcctggtggcaccctcacagagcctgtccatcacatgcaccgtctcaggattctcattaagcggctatggcataagctgggttcgccagcctccaggaaagcgtctggaatggctgggattgatatggggtgatggaaccacagactataattcagctctcaaatccagactgagcatcagcaaggacaactccaagagccaggttttcttaaaaatgaacagtctgcaaactgatgacacagccaggtacttctgtaccagagggcctccggccttctataagtacctctactttgactactggggccaaggcaccactctcacagtctcctcagacaaaactcacacatgcccaccgtgcccagcacctcctgtggcaggaccgtcagtcttcctcttccccccaaaacccaaggacaccctcatgatctcccggacccctgaggtcacatgcgtggtggtggacgtgagccacgaagaccctgaggtcaagttcaactggtacgtggacggcgtggaggtgcataatgccaagacaaagccgcgggaggagcagtaccagagcacgtaccgtgtggtcagcgtcctcaccgtcctgcaccaggactggctgaatggcaaggagtacaagtgcaaggtctccaacaaagccctcccagcccccatcgagaaaaccatctccaaagccaaagggcagccccgagaaccacaggtgtacaccctgccaccatcacgagatgagctgaccaagaaccaggtcagcctgacctgcctggtcaaaggcttctatcccagcgacatcgccgtggagtgggagagcaatgggcagccggagaacaactacaagaccacgcctcccgtgctggactccgacggctccttcttcctctacagcaagctcaccgtggacaagagcaggtggcagcaggggaacgtcttctcatgctccgtgatgcatgaggctctgcacaaccactacacgcagaagagcctctccctgtctcccttttgggtgctggtggtggttggtggagtcctggcttgctatagcttgctagtaacagtggcctttattattttctgggtgaggagtaagaggagcaggggaggtcacagtgactacatgaacatgactccccgccgccccgggcccacccgcaagcattaccagccctatgccccaccacgcgacttcgcagcctatcgctccaaacggggcagaaagaaactcctgtatatattcaaacaaccatttatgagaccagtacaaactactcaagaggaagatggctgtagctgccgatttccagaagaagaagaaggaggatgtgaactgagagtgaagttcagcaggagcgcagacgcccccgcgtaccagcagggccagaaccagctctataacgagctcaatctaggacgaagagaggagtacgatgttttggacaagagacgtggccgggaccctgagatggggggaaagccgagaaggaagaaccctcaggaaggcctgtacaatgaactgcagaaagataagatggcggaggcctacagtgagattgggatgaaaggcgagcgccggaggggcaaggggcacgatggcctttaccagggtctcagtacagccaccaaggacacctacgacgcccttcacatgcaggccctgccccctcgccagtgtactaattatgctctcttgaaattggctggagatgttgagagcaaccccgggccgatgcccaaccctaggccagccaagcctatggctccttccttggcccttggcccatccccaggagtcttgccaagctggaagactgcacccaagggctcagaacttctagggaccaggggctctgggggacccttccaaggtcgggacctgcgaagtggggcccacacctcttcttccttgaaccccctgccaccatcccagctgcagctgcctacagtgcccctagtcatggtggcaccgtctggggcccgactaggtccctcaccccacctacaggcccttctccaggacagaccacacttcatgcatcagctctccactgtggatgcccatgcccagacccctgtgctccaagtgcgtccactggacaacccagccatgatcagcctcccaccaccttctgctgccactggggtcttctccctcaaggcccggcctggcctgccacctgggatcaatgtggccagtctggaatgggtgtccagggagccagctctactctgcaccttcccacgctcgggtacacccaggaaagacagcaaccttttggctgcaccccaaggatcctacccactgctggcaaatggagtctgcaagtggcctggttgtgagaaggtcttcgaggagccagaagagtttctcaagcactgccaagcagatcatctcctggatgagaaaggcaaggcccagtgcctcctccagagagaagtggtgcagtctctggagcagcagctggagctggaaaaggagaagctgggagctatgcaggcccacctggctgggaagatggcgctggccaaggctccatctgtggcctcaatggacaagagctcttgctgcatcgtagccaccagtactcagggcagtgtgctcccggcctggtctgctcctcgggaggctccagacggcggcctgtttgcagtgcggaggcacctctggggaagccatggcaatagttccttcccagagttcttccacaacatggactacttcaagtaccacaatatgcgaccccctttcacctatgccacccttatccgatgggccatcctggaagccccggagaggcagaggacactcaatgaaatctaccattggtttactcgcatgttcgcctacttcagaaaccaccccgccacctggaagaatgccatccgccacaacctgagcctgcacaagtgctttgtgcgagtggagagcgagaagggagcagtgtggaccgtagatgaatttgagtttcgcaagaagaggagccaacgccccaacaagtgctccaatccctgcccttgaaattcgagcatcttaccgccatttattcccatatttgttctgtttttcttgatttgggtatacatttaaatgttaataaaacaaaatggtggggcaatcatttacatttttagggatatgtaattactagttcaggtgtattgccacaagacaaacatgttaagaaactttcccgttatttacgctctgttcctgttaatcaacctctggattacaaaatttgtgaaagattgactgatattcttaactatgttgctccttttacgctgtgtggatatgctgctttatagcctctgtatctagctattgcttcccgtacggctttcgttttctcctccttgtataaatcctggttgctgtctcttttagaggagttgtggcccgttgtccgtcaacgtggcgtggtgtgctctgtgtttgctgacgcaacccccactggctggggcattgccaccacctgtcaactcctttctgggactttcgctttccccctcccgatcgccacggcagaactcatcgccgcctgccttgcccgctgctggacaggggctaggttgctgggcactgataattccgtggtgttgtcggggaagctgacgtcctttcctcgagggggggcccggtacctttaagaccaatgacttacaaggcagctgtagatcttagccactttttaaaagaaaaggggggactggaagggctaattcactcccaacgaagacaagatctgctttttgcttgtactgggtctctctggttagaccagatctgagcctgggagctctctggctaactagggaacccactgcttaagcctcaataaagcttgccttgagtgcttcaagtagtgtgtgcccgtctgttgtgtgactctggtaactagagatccctcagacccttttagtcagtgtggaaaatctctagcagtagtagttcatgtcatcttattattcagtatttataacttgcaaagaaatgaatatcagagagtgagaggaacttgtttattgcagcttataatggttacaaataaagcaatagcatcacaaatttcacaaataaagcatttttttcactgcattctagttgtggtttgtccaaactcatcaatgtatcttatcatgtctggctctagctatcccgcccctaactccgcccagttccgcccattctccgccccatggctgactaattttttttatttatgcagaggccgaggccgcctcggcctctgagctattccagaagtagtgaggaggcttttttggaggcctaggcttttgcgtcgagacgtacccaattcgccctatagtgagtcgtattacgcgcgctcactggccgtcgttttacaacgtcgtgactgggaaaaccctggcgttacccaacttaatcgccttgcagcacatccccctttcgccagctggcgtaatagcgaagaggcccgcaccgatcgcccttcccaacagttgcgcagcctgaatggcgaatggcgcgacgcgccctgtagcggcgcattaagcgcggcgggtgtggtggttacgcgcagcgtgaccgctacacttgccagcgccctagcgcccgctcctttcgctttcttcccttcctttctcgccacgttcgccggctttccccgtcaagctctaaatcgggggctccctttagggttccgatttagtgctttacggcacctcgaccccaaaaaacttgattagggtgatggttcacgtagtgggccatcgccctgatagacggtttttcgccctttgacgttggagtccacgttctttaatagtggactcttgttccaaactggaacaacactcaaccctatctcggtctattcttttgatttataagggattttgccgatttcggcctattggttaaaaaatgagctgatttaacaaaaatttaacgcgaattttaacaaaatattaacgtttacaatttcccaggtggcacttttcggggaaatgtgcgcggaacccctatttgtttatttttctaaatacattcaaatatgtatccgctcatgagacaataaccctgataaatgcttcaataatattgaaaaaggaagagtatgagtattcaacatttccgtgtcgcccttattcccttttttgcggcattttgccttcctgtttttgctcacccagaaacgctggtgaaagtaaaagatgctgaagatcagttgggtgcacgagtgggttacatcgaactggatctcaacagcggtaagatccttgagagttttcgccccgaagaacgttttccaatgatgagcacttttaaagttctgctatgtggcgcggtattatcccgtattgacgccgggcaagagcaactcggtcgccgcatacactattctcagaatgacttggttgagtactcaccagtcacagaaaagcatcttacggatggcatgacagtaagagaattatgcagtgctgccataaccatgagtgataacactgcggccaacttacttctgacaacgatcggaggaccgaaggagctaaccgcttttttgcacaacatgggggatcatgtaactcgccttgatcgttgggaaccggagctgaatgaagccataccaaacgacgagcgtgacaccacgatgcctgtagcaatggcaacaacgttgcgcaaactattaactggcgaactacttactctagcttcccggcaacaattaatagactggatggaggcggataaagttgcaggaccacttctgcgctcggcccttccggctggctggtttattgctgataaatctggagccggtgagcgtgggtctcgcggtatcattgcagcactggggccagatggtaagccctcccgtatcgtagttatctacacgacggggagtcaggcaactatggatgaacgaaatagacagatcgctgagataggtgcctcactgattaagcattggtaactgtcagaccaagtttactcatatatactttagattgatttaaaacttcatttttaatttaaaaggatctaggtgaagatcctttttgataatctcatgaccaaaatcccttaacgtgagttttcgttccactgagcgtcagaccccgtagaaaagatcaaaggatcttcttgagatcctttttttctgcgcgtaatctgctgcttgcaaacaaaaaaaccaccgctaccagcggtggtttgtttgccggatcaagagctaccaactctttttccgaaggtaactggcttcagcagagcgcagataccaaatactgtccttctagtgtagccgtagttaggccaccacttcaagaactctgtagcaccgcctacatacctcgctctgctaatcctgttaccagtggctgctgccagtggcgataagtcgtgtcttaccgggttggactcaagacgatagttaccggataaggcgcagcggtcgggctgaacggggggttcgtgcacacagcccagcttggagcgaacgacctacaccgaactgagatacctacagcgtgagctatgagaaagcgccacgcttcccgaagggagaaaggcggacaggtatccggtaagcggcagggtcggaacaggagagcgcacgagggagcttccagggggaaacgcctggtatctttatagtcctgtcgggtttcgccacctctgacttgagcgtcgatttttgtgatgctcgtcaggggggcggagcctatggaaaaacgccagcaacgcggcctttttacggttcctggccttttgctggccttttgctcacatgttctttcctgcgttatcccctgattctgtggataaccgtattaccgcctttgagtgagctgataccgctcgccgcagccgaacgaccgagcgcagcgagtcagtgagcgaggaagcggaagagcgcccaatacgcaaaccgcctctccccgcgcgttggccgattcattaatgcagctggcacgacaggtttcccgactggaaagcgggcagtgagcgcaacgcaattaatgtgagttagctcactcattaggcaccccaggctttacactttatgcttccggctcgtatgttgtgtggaattgtgagcggataacaatttcacacaggaaacagctatgaccatgattacgccaagcgcgcaattaaccctcactaaagggaacaaaagctggagctgcaagcttaatgtagtcttatgcaatactcttgtagtcttgcaacatggtaacgatgagttagcaacatgccttacaaggagagaaaaagcaccgtgcatgccgattggtggaagtaaggtggtacgatcgtgccttattaggaaggcaacagacgggtctgacatggattggacgaaccactgaattgccgcattgcagagatattgtatttaagtgcctagctcgatacataaacgggtctctctggttagaccagatctgagcctgggagctctctggctaactagggaacccactgcttaagcctcaataaagcttgccttgagtgcttcaagtagtgtgtgcccgtctgttgtgtgactctggtaactagagatccctcagacccttttagtcagtgtggaaaatctctagcagtggcgcccgaacagggacttgaaagcgaaagggaaaccagaggagctctctcgacgcaggactcggcttgctgaagcgcgcacggcaagaggcgaggggcggcgactggtgagtacgccaaaaattttgactagcggaggctagaaggagagagatgggtgcgagagcgtcagtattaagcgggggagaattagatcgcgatgggaaaaaattcggttaaggccagggggaaagaaaaaatataaattaaaacatatagtatgggcaagcagggagctagaacgattcgcagttaatcctggcctgttagaaacatcagaaggctgtagacaaatactgggacagctacaaccatcccttcagacaggatcagaagaacttagatcattatataatacagtagcaaccctctattgtgtgcatcaaaggatagagataaaagacaccaaggaagctttagacaagatagaggaagagcaaaacaaaagtaagaccaccgcacagcaagcggccgctgatcttcagacctggaggaggagatatgagggacaattggagaagtgaattatataaatataaagtagtaaaaattgaaccattaggagtagcacccaccaaggcaaagagaagagtggtgcagagagaaaaaagagcagtgggaataggagctttgttccttgggttcttgggagcagcaggaagcactatgggcgcagcctcaatgacgctgacggtacaggccagacaattattgtctggtatagtgcagcagcagaacaatttgctgagggctattgaggcgcaacagcatctgttgcaactcacagtctggggcatcaagcagctccaggcaagaatcctggctgtggaaagatacctaaaggatcaacagctcctggggatttggggttgctctggaaaactcatttgcaccactgctgtgccttggaatgctagttggagtaataaatctctggaacagatttggaatcacacgacctggatggagtgggacagagaaattaacaattacacaagcttaatacactccttaattgaagaatcgcaaaaccagcaagaaaagaatgaacaagaattattggaattagataaatgggcaagtttgtggaattggtttaacataacaaattggctgtggtatataaaattattcataatgatagtaggaggcttggtaggtttaagaatagtttttgctgtactttctatagtgaatagagttaggcagggatattcaccattatcgtttcagacccacctcccaaccccgaggggacccgacaggcccgaaggaatagaagaagaaggtggagagagagacagagacagatccattcgattagtgaacggatctcgacggtatcggtt

SEQ ID NO: 3 - DNA, 9836 bp, Unknown
  CD8leader-AAV-CAR-2A-EGFRt
ctgttttaaaagaaaaggggggattggggggtacagtgcaggggaaagaatagtagacataatagcaacagacatacaaactaaagaattacaaaaacaaattacaaaaattcaaaattttatcaacaagcttgatcgatggctccggtgcccgtcagtgggcagagcgcacatcgcccacagtccccgagaagttggggggaggggtcggcaattgaaccggtgcctagagaaggtggcgcggggtaaactgggaaagtgatgtcgtgtactggctccgcctttttcccgagggtgggggagaaccgtatataagtgcagtagtcgccgtgaacgttctttttcgcaacgggtttgccgccagaacacaggtgtcgtgacgcggatccacgcgtgcggccgcacgcgtaagcttagcgcagaggcttggggcagccgagcggcagccaggccccggcccgggcctcggttccagaagggagaggagcccgccaaggcgcgcaagagagcgggctgcctcgcagtccgagccggagagggagcgcgagccgcgccggccccggacggcctcgccgccaccatggctctgcccgtcaccgcactgctgctgcctctggctctgctgctgcacgccgcaagaccagacattgtgctgacacagtctcctgcttccttagctgtatctctggggcagagggccaccatctcatgcagggccagccaaagtgtcagttcatctacctataattttatacactggtatcaacagaaatcaggacagccacccaaactcctcatcaagtatgcatccaacctagaatctggggtccctgtcaggttcagtggcagtgggtctgggacagacttctccctcaacatccatcctgtggaggaggaggatactgcaacatattactgtcagcacagttgggagattccatacacgttcggagggggggccaagttggagataaaaggcagtactagcggtggtggctccgggggcggttccggtgggggcggcagcagccaggtgcagctgaaggagtcaggacctggcctggtggcaccctcacagagcctgtccatcacatgcaccgtctcaggattctcattaagcggctatggcataagctgggttcgccagcctccaggaaagcgtctggaatggctgggattgatatggggtgatggaaccacagactataattcagctctcaaatccagactgagcatcagcaaggacaactccaagagccaggttttcttaaaaatgaacagtctgcaaactgatgacacagccaggtacttctgtaccagagggcctccggccttctataagtacctctactttgactactggggccaaggcaccactctcacagtctcctcagacaaaactcacacatgcccaccgtgcccagcacctcctgtggcaggaccgtcagtcttcctcttccccccaaaacccaaggacaccctcatgatctcccggacccctgaggtcacatgcgtggtggtggacgtgagccacgaagaccctgaggtcaagttcaactggtacgtggacggcgtggaggtgcataatgccaagacaaagccgcgggaggagcagtaccagagcacgtaccgtgtggtcagcgtcctcaccgtcctgcaccaggactggctgaatggcaaggagtacaagtgcaaggtctccaacaaagccctcccagcccccatcgagaaaaccatctccaaagccaaagggcagccccgagaaccacaggtgtacaccctgccaccatcacgagatgagctgaccaagaaccaggtcagcctgacctgcctggtcaaaggcttctatcccagcgacatcgccgtggagtgggagagcaatgggcagccggagaacaactacaagaccacgcctcccgtgctggactccgacggctccttcttcctctacagcaagctcaccgtggacaagagcaggtggcagcaggggaacgtcttctcatgctccgtgatgcatgaggctctgcacaaccactacacgcagaagagcctctccctgtctcccttttgggtgctggtggtggttggtggagtcctggcttgctatagcttgctagtaacagtggcctttattattttctgggtgaggagtaagaggagcaggggaggtcacagtgactacatgaacatgactccccgccgccccgggcccacccgcaagcattaccagccctatgccccaccacgcgacttcgcagcctatcgctccaaacggggcagaaagaaactcctgtatatattcaaacaaccatttatgagaccagtacaaactactcaagaggaagatggctgtagctgccgatttccagaagaagaagaaggaggatgtgaactgagagtgaagttcagcaggagcgcagacgcccccgcgtaccagcagggccagaaccagctctataacgagctcaatctaggacgaagagaggagtacgatgttttggacaagagacgtggccgggaccctgagatggggggaaagccgagaaggaagaaccctcaggaaggcctgtacaatgaactgcagaaagataagatggcggaggcctacagtgagattgggatgaaaggcgagcgccggaggggcaaggggcacgatggcctttaccagggtctcagtacagccaccaaggacacctacgacgcccttcacatgcaggccctgccccctcgccagtgtactaattatgctctcttgaaattggctggagatgttgagagcaaccccgggccgatgcttctcctggtgacaagccttctgctctgtgagttaccacacccagcattcctcctgatcccacgcaaagtgtgtaacggaataggtattggtgaatttaaagactcactctccataaatgctacgaatattaaacacttcaaaaactgcacctccatcagtggcgatctccacatcctgccggtggcatttaggggtgactccttcacacatactcctcctctggatccacaggaactggatattctgaaaaccgtaaaggaaatcacagggtttttgctgattcaggcttggcctgaaaacaggacggacctccatgcctttgagaacctagaaatcatacgcggcaggaccaagcaacatggtcagttttctcttgcagtcgtcagcctgaacataacatccttgggattacgctccctcaaggagataagtgatggagatgtgataatttcaggaaacaaaaatttgtgctatgcaaatacaataaactggaaaaaactgtttgggacctccggtcagaaaaccaaaattataagcaacagaggtgaaaacagctgcaaggccacaggccaggtctgccatgccttgtgctcccccgagggctgctggggcccggagcccagggactgcgtctcttgccggaatgtcagccgaggcagggaatgcgtggacaagtgcaaccttctggagggtgagccaagggagtttgtggagaactctgagtgcatacagtgccacccagagtgcctgcctcaggccatgaacatcacctgcacaggacggggaccagacaactgtatccagtgtgcccactacattgacggcccccactgcgtcaagacctgcccggcaggagtcatgggagaaaacaacaccctggtctggaagtacgcagacgccggccatgtgtgccacctgtgccatccaaactgcacctacggatgcactgggccaggtcttgaaggctgtccaacgaatgggcctaagatcccgtccatcgccactgggatggtgggggccctcctcttgctgctggtggtggccctggggatcggcctcttcatgtgaggaattcgagcatcttaccgccatttattcccatatttgttctgtttttcttgatttgggtatacatttaaatgttaataaaacaaaatggtggggcaatcatttacatttttagggatatgtaattactagttcaggtgtattgccacaagacaaacatgttaagaaactttcccgttatttacgctctgttcctgttaatcaacctctggattacaaaatttgtgaaagattgactgatattcttaactatgttgctccttttacgctgtgtggatatgctgctttatagcctctgtatctagctattgcttcccgtacggctttcgttttctcctccttgtataaatcctggttgctgtctcttttagaggagttgtggcccgttgtccgtcaacgtggcgtggtgtgctctgtgtttgctgacgcaacccccactggctggggcattgccaccacctgtcaactcctttctgggactttcgctttccccctcccgatcgccacggcagaactcatcgccgcctgccttgcccgctgctggacaggggctaggttgctgggcactgataattccgtggtgttgtcggggaagctgacgtcctttcctcgagggggggcccggtacctttaagaccaatgacttacaaggcagctgtagatcttagccactttttaaaagaaaaggggggactggaagggctaattcactcccaacgaagacaagatctgctttttgcttgtactgggtctctctggttagaccagatctgagcctgggagctctctggctaactagggaacccactgcttaagcctcaataaagcttgccttgagtgcttcaagtagtgtgtgcccgtctgttgtgtgactctggtaactagagatccctcagacccttttagtcagtgtggaaaatctctagcagtagtagttcatgtcatcttattattcagtatttataacttgcaaagaaatgaatatcagagagtgagaggaacttgtttattgcagcttataatggttacaaataaagcaatagcatcacaaatttcacaaataaagcatttttttcactgcattctagttgtggtttgtccaaactcatcaatgtatcttatcatgtctggctctagctatcccgcccctaactccgcccagttccgcccattctccgccccatggctgactaattttttttatttatgcagaggccgaggccgcctcggcctctgagctattccagaagtagtgaggaggcttttttggaggcctaggcttttgcgtcgagacgtacccaattcgccctatagtgagtcgtattacgcgcgctcactggccgtcgttttacaacgtcgtgactgggaaaaccctggcgttacccaacttaatcgccttgcagcacatccccctttcgccagctggcgtaatagcgaagaggcccgcaccgatcgcccttcccaacagttgcgcagcctgaatggcgaatggcgcgacgcgccctgtagcggcgcattaagcgcggcgggtgtggtggttacgcgcagcgtgaccgctacacttgccagcgccctagcgcccgctcctttcgctttcttcccttcctttctcgccacgttcgccggctttccccgtcaagctctaaatcgggggctccctttagggttccgatttagtgctttacggcacctcgaccccaaaaaacttgattagggtgatggttcacgtagtgggccatcgccctgatagacggtttttcgccctttgacgttggagtccacgttctttaatagtggactcttgttccaaactggaacaacactcaaccctatctcggtctattcttttgatttataagggattttgccgatttcggcctattggttaaaaaatgagctgatttaacaaaaatttaacgcgaattttaacaaaatattaacgtttacaatttcccaggtggcacttttcggggaaatgtgcgcggaacccctatttgtttatttttctaaatacattcaaatatgtatccgctcatgagacaataaccctgataaatgcttcaataatattgaaaaaggaagagtatgagtattcaacatttccgtgtcgcccttattcccttttttgcggcattttgccttcctgtttttgctcacccagaaacgctggtgaaagtaaaagatgctgaagatcagttgggtgcacgagtgggttacatcgaactggatctcaacagcggtaagatccttgagagttttcgccccgaagaacgttttccaatgatgagcacttttaaagttctgctatgtggcgcggtattatcccgtattgacgccgggcaagagcaactcggtcgccgcatacactattctcagaatgacttggttgagtactcaccagtcacagaaaagcatcttacggatggcatgacagtaagagaattatgcagtgctgccataaccatgagtgataacactgcggccaacttacttctgacaacgatcggaggaccgaaggagctaaccgcttttttgcacaacatgggggatcatgtaactcgccttgatcgttgggaaccggagctgaatgaagccataccaaacgacgagcgtgacaccacgatgcctgtagcaatggcaacaacgttgcgcaaactattaactggcgaactacttactctagcttcccggcaacaattaatagactggatggaggcggataaagttgcaggaccacttctgcgctcggcccttccggctggctggtttattgctgataaatctggagccggtgagcgtgggtctcgcggtatcattgcagcactggggccagatggtaagccctcccgtatcgtagttatctacacgacggggagtcaggcaactatggatgaacgaaatagacagatcgctgagataggtgcctcactgattaagcattggtaactgtcagaccaagtttactcatatatactttagattgatttaaaacttcatttttaatttaaaaggatctaggtgaagatcctttttgataatctcatgaccaaaatcccttaacgtgagttttcgttccactgagcgtcagaccccgtagaaaagatcaaaggatcttcttgagatcctttttttctgcgcgtaatctgctgcttgcaaacaaaaaaaccaccgctaccagcggtggtttgtttgccggatcaagagctaccaactctttttccgaaggtaactggcttcagcagagcgcagataccaaatactgtccttctagtgtagccgtagttaggccaccacttcaagaactctgtagcaccgcctacatacctcgctctgctaatcctgttaccagtggctgctgccagtggcgataagtcgtgtcttaccgggttggactcaagacgatagttaccggataaggcgcagcggtcgggctgaacggggggttcgtgcacacagcccagcttggagcgaacgacctacaccgaactgagatacctacagcgtgagctatgagaaagcgccacgcttcccgaagggagaaaggcggacaggtatccggtaagcggcagggtcggaacaggagagcgcacgagggagcttccagggggaaacgcctggtatctttatagtcctgtcgggtttcgccacctctgacttgagcgtcgatttttgtgatgctcgtcaggggggcggagcctatggaaaaacgccagcaacgcggcctttttacggttcctggccttttgctggccttttgctcacatgttctttcctgcgttatcccctgattctgtggataaccgtattaccgcctttgagtgagctgataccgctcgccgcagccgaacgaccgagcgcagcgagtcagtgagcgaggaagcggaagagcgcccaatacgcaaaccgcctctccccgcgcgttggccgattcattaatgcagctggcacgacaggtttcccgactggaaagcgggcagtgagcgcaacgcaattaatgtgagttagctcactcattaggcaccccaggctttacactttatgcttccggctcgtatgttgtgtggaattgtgagcggataacaatttcacacaggaaacagctatgaccatgattacgccaagcgcgcaattaaccctcactaaagggaacaaaagctggagctgcaagcttaatgtagtcttatgcaatactcttgtagtcttgcaacatggtaacgatgagttagcaacatgccttacaaggagagaaaaagcaccgtgcatgccgattggtggaagtaaggtggtacgatcgtgccttattaggaaggcaacagacgggtctgacatggattggacgaaccactgaattgccgcattgcagagatattgtatttaagtgcctagctcgatacataaacgggtctctctggttagaccagatctgagcctgggagctctctggctaactagggaacccactgcttaagcctcaataaagcttgccttgagtgcttcaagtagtgtgtgcccgtctgttgtgtgactctggtaactagagatccctcagacccttttagtcagtgtggaaaatctctagcagtggcgcccgaacagggacttgaaagcgaaagggaaaccagaggagctctctcgacgcaggactcggcttgctgaagcgcgcacggcaagaggcgaggggcggcgactggtgagtacgccaaaaattttgactagcggaggctagaaggagagagatgggtgcgagagcgtcagtattaagcgggggagaattagatcgcgatgggaaaaaattcggttaaggccagggggaaagaaaaaatataaattaaaacatatagtatgggcaagcagggagctagaacgattcgcagttaatcctggcctgttagaaacatcagaaggctgtagacaaatactgggacagctacaaccatcccttcagacaggatcagaagaacttagatcattatataatacagtagcaaccctctattgtgtgcatcaaaggatagagataaaagacaccaaggaagctttagacaagatagaggaagagcaaaacaaaagtaagaccaccgcacagcaagcggccgctgatcttcagacctggaggaggagatatgagggacaattggagaagtgaattatataaatataaagtagtaaaaattgaaccattaggagtagcacccaccaaggcaaagagaagagtggtgcagagagaaaaaagagcagtgggaataggagctttgttccttgggttcttgggagcagcaggaagcactatgggcgcagcctcaatgacgctgacggtacaggccagacaattattgtctggtatagtgcagcagcagaacaatttgctgagggctattgaggcgcaacagcatctgttgcaactcacagtctggggcatcaagcagctccaggcaagaatcctggctgtggaaagatacctaaaggatcaacagctcctggggatttggggttgctctggaaaactcatttgcaccactgctgtgccttggaatgctagttggagtaataaatctctggaacagatttggaatcacacgacctggatggagtgggacagagaaattaacaattacacaagcttaatacactccttaattgaagaatcgcaaaaccagcaagaaaagaatgaacaagaattattggaattagataaatgggcaagtttgtggaattggtttaacataacaaattggctgtggtatataaaattattcataatgatagtaggaggcttggtaggtttaagaatagtttttgctgtactttctatagtgaatagagttaggcagggatattcaccattatcgtttcagacccacctcccaaccccgaggggacccgacaggcccgaaggaatagaagaagaaggtggagagagagacagagacagatccattcgattagtgaacggatctcgacggtatcggtt

SEQ ID NO: 4 - DNA, 8711 bp, Unknown
  13-1_Lenti-IF5-D3-NQ-28-BB-Z
ctgttttaaaagaaaaggggggattggggggtacagtgcaggggaaagaatagtagacataatagcaacagacatacaaactaaagaattacaaaaacaaattacaaaaattcaaaattttatcaacaagcttgatcgatggctccggtgcccgtcagtgggcagagcgcacatcgcccacagtccccgagaagttggggggaggggtcggcaattgaaccggtgcctagagaaggtggcgcggggtaaactgggaaagtgatgtcgtgtactggctccgcctttttcccgagggtgggggagaaccgtatataagtgcagtagtcgccgtgaacgttctttttcgcaacgggtttgccgccagaacacaggtgtcgtgacgcggatccacgcgtgcggccgcacgcgtaagcttagcgcagaggcttggggcagccgagcggcagccaggccccggcccgggcctcggttccagaagggagaggagcccgccaaggcgcgcaagagagcgggctgcctcgcagtccgagccggagagggagcgcgagccgcgccggccccggacggcctcgccgccaccatggagacagacacactcctgctatgggtgctgctgctctgggttccaggttccactggtgacattgtgctgacacagtctcctgcttccttagctgtatctctggggcagagggccaccatctcatgcagggccagccaaagtgtcagttcatctacctataattttatacactggtatcaacagaaatcaggacagccacccaaactcctcatcaagtatgcatccaacctagaatctggggtccctgtcaggttcagtggcagtgggtctgggacagacttctccctcaacatccatcctgtggaggaggaggatactgcaacatattactgtcagcacagttgggagattccatacacgttcggagggggggccaagttggagataaaaggcagtactagcggtggtggctccgggggcggttccggtgggggcggcagcagccaggtgcagctgaaggagtcaggacctggcctggtggcaccctcacagagcctgtccatcacatgcaccgtctcaggattctcattaagcggctatggcataagctgggttcgccagcctccaggaaagcgtctggaatggctgggattgatatggggtgatggaaccacagactataattcagctctcaaatccagactgagcatcagcaaggacaactccaagagccaggttttcttaaaaatgaacagtctgcaaactgatgacacagccaggtacttctgtaccagagggcctccggccttctataagtacctctactttgactactggggccaaggcaccactctcacagtctcctcagacaaaactcacacatgcccaccgtgcccagcacctcctgtggcaggaccgtcagtcttcctcttccccccaaaacccaaggacaccctcatgatctcccggacccctgaggtcacatgcgtggtggtggacgtgagccacgaagaccctgaggtcaagttcaactggtacgtggacggcgtggaggtgcataatgccaagacaaagccgcgggaggagcagtaccagagcacgtaccgtgtggtcagcgtcctcaccgtcctgcaccaggactggctgaatggcaaggagtacaagtgcaaggtctccaacaaagccctcccagcccccatcgagaaaaccatctccaaagccaaagggcagccccgagaaccacaggtgtacaccctgccaccatcacgagatgagctgaccaagaaccaggtcagcctgacctgcctggtcaaaggcttctatcccagcgacatcgccgtggagtgggagagcaatgggcagccggagaacaactacaagaccacgcctcccgtgctggactccgacggctccttcttcctctacagcaagctcaccgtggacaagagcaggtggcagcaggggaacgtcttctcatgctccgtgatgcatgaggctctgcacaaccactacacgcagaagagcctctccctgtctcccttttgggtgctggtggtggttggtggagtcctggcttgctatagcttgctagtaacagtggcctttattattttctgggtgaggagtaagaggagcaggggaggtcacagtgactacatgaacatgactccccgccgccccgggcccacccgcaagcattaccagccctatgccccaccacgcgacttcgcagcctatcgctccaaacggggcagaaagaaactcctgtatatattcaaacaaccatttatgagaccagtacaaactactcaagaggaagatggctgtagctgccgatttccagaagaagaagaaggaggatgtgaactgagagtgaagttcagcaggagcgcagacgcccccgcgtaccagcagggccagaaccagctctataacgagctcaatctaggacgaagagaggagtacgatgttttggacaagagacgtggccgggaccctgagatggggggaaagccgagaaggaagaaccctcaggaaggcctgtacaatgaactgcagaaagataagatggcggaggcctacagtgagattgggatgaaaggcgagcgccggaggggcaaggggcacgatggcctttaccagggtctcagtacagccaccaaggacacctacgacgcccttcacatgcaggccctgccccctcgctgagatatcgtgggaattcgagcatcttaccgccatttattcccatatttgttctgtttttcttgatttgggtatacatttaaatgttaataaaacaaaatggtggggcaatcatttacatttttagggatatgtaattactagttcaggtgtattgccacaagacaaacatgttaagaaactttcccgttatttacgctctgttcctgttaatcaacctctggattacaaaatttgtgaaagattgactgatattcttaactatgttgctccttttacgctgtgtggatatgctgctttatagcctctgtatctagctattgcttcccgtacggctttcgttttctcctccttgtataaatcctggttgctgtctcttttagaggagttgtggcccgttgtccgtcaacgtggcgtggtgtgctctgtgtttgctgacgcaacccccactggctggggcattgccaccacctgtcaactcctttctgggactttcgctttccccctcccgatcgccacggcagaactcatcgccgcctgccttgcccgctgctggacaggggctaggttgctgggcactgataattccgtggtgttgtcggggaagctgacgtcctttcctcgagggggggcccggtacctttaagaccaatgacttacaaggcagctgtagatcttagccactttttaaaagaaaaggggggactggaagggctaattcactcccaacgaagacaagatctgctttttgcttgtactgggtctctctggttagaccagatctgagcctgggagctctctggctaactagggaacccactgcttaagcctcaataaagcttgccttgagtgcttcaagtagtgtgtgcccgtctgttgtgtgactctggtaactagagatccctcagacccttttagtcagtgtggaaaatctctagcagtagtagttcatgtcatcttattattcagtatttataacttgcaaagaaatgaatatcagagagtgagaggaacttgtttattgcagcttataatggttacaaataaagcaatagcatcacaaatttcacaaataaagcatttttttcactgcattctagttgtggtttgtccaaactcatcaatgtatcttatcatgtctggctctagctatcccgcccctaactccgcccagttccgcccattctccgccccatggctgactaattttttttatttatgcagaggccgaggccgcctcggcctctgagctattccagaagtagtgaggaggcttttttggaggcctaggcttttgcgtcgagacgtacccaattcgccctatagtgagtcgtattacgcgcgctcactggccgtcgttttacaacgtcgtgactgggaaaaccctggcgttacccaacttaatcgccttgcagcacatccccctttcgccagctggcgtaatagcgaagaggcccgcaccgatcgcccttcccaacagttgcgcagcctgaatggcgaatggcgcgacgcgccctgtagcggcgcattaagcgcggcgggtgtggtggttacgcgcagcgtgaccgctacacttgccagcgccctagcgcccgctcctttcgctttcttcccttcctttctcgccacgttcgccggctttccccgtcaagctctaaatcgggggctccctttagggttccgatttagtgctttacggcacctcgaccccaaaaaacttgattagggtgatggttcacgtagtgggccatcgccctgatagacggtttttcgccctttgacgttggagtccacgttctttaatagtggactcttgttccaaactggaacaacactcaaccctatctcggtctattcttttgatttataagggattttgccgatttcggcctattggttaaaaaatgagctgatttaacaaaaatttaacgcgaattttaacaaaatattaacgtttacaatttcccaggtggcacttttcggggaaatgtgcgcggaacccctatttgtttatttttctaaatacattcaaatatgtatccgctcatgagacaataaccctgataaatgcttcaataatattgaaaaaggaagagtatgagtattcaacatttccgtgtcgcccttattcccttttttgcggcattttgccttcctgtttttgctcacccagaaacgctggtgaaagtaaaagatgctgaagatcagttgggtgcacgagtgggttacatcgaactggatctcaacagcggtaagatccttgagagttttcgccccgaagaacgttttccaatgatgagcacttttaaagttctgctatgtggcgcggtattatcccgtattgacgccgggcaagagcaactcggtcgccgcatacactattctcagaatgacttggttgagtactcaccagtcacagaaaagcatcttacggatggcatgacagtaagagaattatgcagtgctgccataaccatgagtgataacactgcggccaacttacttctgacaacgatcggaggaccgaaggagctaaccgcttttttgcacaacatgggggatcatgtaactcgccttgatcgttgggaaccggagctgaatgaagccataccaaacgacgagcgtgacaccacgatgcctgtagcaatggcaacaacgttgcgcaaactattaactggcgaactacttactctagcttcccggcaacaattaatagactggatggaggcggataaagttgcaggaccacttctgcgctcggcccttccggctggctggtttattgctgataaatctggagccggtgagcgtgggtctcgcggtatcattgcagcactggggccagatggtaagccctcccgtatcgtagttatctacacgacggggagtcaggcaactatggatgaacgaaatagacagatcgctgagataggtgcctcactgattaagcattggtaactgtcagaccaagtttactcatatatactttagattgatttaaaacttcatttttaatttaaaaggatctaggtgaagatcctttttgataatctcatgaccaaaatcccttaacgtgagttttcgttccactgagcgtcagaccccgtagaaaagatcaaaggatcttcttgagatcctttttttctgcgcgtaatctgctgcttgcaaacaaaaaaaccaccgctaccagcggtggtttgtttgccggatcaagagctaccaactctttttccgaaggtaactggcttcagcagagcgcagataccaaatactgtccttctagtgtagccgtagttaggccaccacttcaagaactctgtagcaccgcctacatacctcgctctgctaatcctgttaccagtggctgctgccagtggcgataagtcgtgtcttaccgggttggactcaagacgatagttaccggataaggcgcagcggtcgggctgaacggggggttcgtgcacacagcccagcttggagcgaacgacctacaccgaactgagatacctacagcgtgagctatgagaaagcgccacgcttcccgaagggagaaaggcggacaggtatccggtaagcggcagggtcggaacaggagagcgcacgagggagcttccagggggaaacgcctggtatctttatagtcctgtcgggtttcgccacctctgacttgagcgtcgatttttgtgatgctcgtcaggggggcggagcctatggaaaaacgccagcaacgcggcctttttacggttcctggccttttgctggccttttgctcacatgttctttcctgcgttatcccctgattctgtggataaccgtattaccgcctttgagtgagctgataccgctcgccgcagccgaacgaccgagcgcagcgagtcagtgagcgaggaagcggaagagcgcccaatacgcaaaccgcctctccccgcgcgttggccgattcattaatgcagctggcacgacaggtttcccgactggaaagcgggcagtgagcgcaacgcaattaatgtgagttagctcactcattaggcaccccaggctttacactttatgcttccggctcgtatgttgtgtggaattgtgagcggataacaatttcacacaggaaacagctatgaccatgattacgccaagcgcgcaattaaccctcactaaagggaacaaaagctggagctgcaagcttaatgtagtcttatgcaatactcttgtagtcttgcaacatggtaacgatgagttagcaacatgccttacaaggagagaaaaagcaccgtgcatgccgattggtggaagtaaggtggtacgatcgtgccttattaggaaggcaacagacgggtctgacatggattggacgaaccactgaattgccgcattgcagagatattgtatttaagtgcctagctcgatacataaacgggtctctctggttagaccagatctgagcctgggagctctctggctaactagggaacccactgcttaagcctcaataaagcttgccttgagtgcttcaagtagtgtgtgcccgtctgttgtgtgactctggtaactagagatccctcagacccttttagtcagtgtggaaaatctctagcagtggcgcccgaacagggacttgaaagcgaaagggaaaccagaggagctctctcgacgcaggactcggcttgctgaagcgcgcacggcaagaggcgaggggcggcgactggtgagtacgccaaaaattttgactagcggaggctagaaggagagagatgggtgcgagagcgtcagtattaagcgggggagaattagatcgcgatgggaaaaaattcggttaaggccagggggaaagaaaaaatataaattaaaacatatagtatgggcaagcagggagctagaacgattcgcagttaatcctggcctgttagaaacatcagaaggctgtagacaaatactgggacagctacaaccatcccttcagacaggatcagaagaacttagatcattatataatacagtagcaaccctctattgtgtgcatcaaaggatagagataaaagacaccaaggaagctttagacaagatagaggaagagcaaaacaaaagtaagaccaccgcacagcaagcggccgctgatcttcagacctggaggaggagatatgagggacaattggagaagtgaattatataaatataaagtagtaaaaattgaaccattaggagtagcacccaccaaggcaaagagaagagtggtgcagagagaaaaaagagcagtgggaataggagctttgttccttgggttcttgggagcagcaggaagcactatgggcgcagcctcaatgacgctgacggtacaggccagacaattattgtctggtatagtgcagcagcagaacaatttgctgagggctattgaggcgcaacagcatctgttgcaactcacagtctggggcatcaagcagctccaggcaagaatcctggctgtggaaagatacctaaaggatcaacagctcctggggatttggggttgctctggaaaactcatttgcaccactgctgtgccttggaatgctagttggagtaataaatctctggaacagatttggaatcacacgacctggatggagtgggacagagaaattaacaattacacaagcttaatacactccttaattgaagaatcgcaaaaccagcaagaaaagaatgaacaagaattattggaattagataaatgggcaagtttgtggaattggtttaacataacaaattggctgtggtatataaaattattcataatgatagtaggaggcttggtaggtttaagaatagtttttgctgtactttctatagtgaatagagttaggcagggatattcaccattatcgtttcagacccacctcccaaccccgaggggacccgacaggcccgaaggaatagaagaagaaggtggagagagagacagagacagatccattcgattagtgaacggatctcgacggtatcggtt

SEQ ID NO: 5 - DNA, 5054 bp, Unknown
  EF1alpha
gtcgacattgattattgactagatcatcgcgtgaggctccggtgcccgtcagtgggcagagcgcacatcgcccacagtccccgagaagttggggggaggggtcggcaattgaaccggtgcctagagaaggtggcgcggggtaaactgggaaagtgatgtcgtgtactggctccgcctttttcccgagggtgggggagaaccgtatataagtgcagtagtcgccgtgaacgttctttttcgcaacgggtttgccgccagaacacaggtaagtgccgtgtgtggttcccgcgggcctggcctctttacgggttatggcccttgcgtgccttgaattacttccacgcccctggctgcagtacgtgattcttgatcccgagcttcgggttggaagtgggtgggagagttcgaggccttgcgcttaaggagccccttcgcctcgtgcttgagttgaggcctggcctgggcgctggggccgccgcgtgcgaatctggtggcaccttcgcgcctgtctcgctgctttcgataagtctctagccatttaaaatttttgatgacctgctgcgacgctttttttctggcaagatagtcttgtaaatgcgggccaagatctgcacactggtatttcggtttttggggccgcgggcggcgacggggcccgtgcgtcccagcgcacatgttcggcgaggcggggcctgcgagcgcggccaccgagaatcggacgggggtagtctcaagctggccggcctgctctggtgcctggcctcgcgccgccgtgtatcgccccgccctgggcggcaaggctggcccggtcggcaccagttgcgtgagcggaaagatggccgcttcccggccctgctgcagggagctcaaaatggaggacgcggcgctcgggagagcgggcgggtgagtcacccacacaaaggaaaagggcctttccgtcctcagccgtcgcttcatgtgactccacggagtaccgggcgccgtccaggcacctcgattagttctcgagcttttggagtacgtcgtctttaggttggggggaggggttttatgcgatggagtttccccacactgagtgggtggagactgaagttaggccagcttggcacttgatgtaattctccttggaatttgccctttttgagtttggatcttggttcattctcaagcctcagacagtggttcaaagtttttttcttccatttcaggtgtcgtgaggaattctgcagtcgacggtaccgcgggcccgggatccaccggtcgccaccatggtgagcaagggcgaggagctgttcaccggggtggtgcccatcctggtcgagctggacggcgacgtaaacggccacaagttcagcgtgtccggcgagggcgagggcgatgccacctacggcaagctgaccctgaagttcatctgcaccaccggcaagctgcccgtgccctggcccaccctcgtgaccaccctgacctacggcgtgcagtgcttcagccgctaccccgaccacatgaagcagcacgacttcttcaagtccgccatgcccgaaggctacgtccaggagcgcaccatcttcttcaaggacgacggcaactacaagacccgcgccgaggtgaagttcgagggcgacaccctggtgaaccgcatcgagctgaagggcatcgacttcaaggaggacggcaacatcctggggcacaagctggagtacaactacaacagccacaacgtctatatcatggccgacaagcagaagaacggcatcaaggtgaacttcaagatccgccacaacatcgaggacggcagcgtgcagctcgccgaccactaccagcagaacacccccatcggcgacggccccgtgctgctgcccgacaaccactacctgagcacccagtccgccctgagcaaagaccccaacgagaagcgcgatcacatggtcctgctggagttcgtgaccgccgccgggatcactctcggcatggacgagctgtacaagtaaagcggccgcactcctcaggtgcaggctgcctatcagaaggtggtggctggtgtggccaatgccctggctcacaaataccactgagatctttttccctctgccaaaaattatggggacatcatgaagccccttgagcatctgacttctggctaataaaggaaatttattttcattgcaatagtgtgttggaattttttgtgtctctcactcggaaggacatatgggagggcaaatcatttaaaacatcagaatgagtatttggtttagagtttggcaacatatgcccatatgctggctgccatgaacaaaggttggctataaagaggtcatcagtatatgaaacagccccctgctgtccattccttattccatagaaaagccttgacttgaggttagattttttttatattttgttttgtgttatttttttctttaacatccctaaaattttccttacatgttttactagccagatttttcctcctctcctgactactcccagtcatagctgtccctcttctcttatggagatccctcgacctgcagcccaagcttggcgtaatcatggtcatagctgtttcctgtgtgaaattgttatccgctcacaattccacacaacatacgagccggaagcataaagtgtaaagcctggggtgcctaatgagtgagctaactcacattaattgcgttgcgctcactgcccgctttccagtcgggaaacctgtcgtgccagcggatccgcatctcaattagtcagcaaccatagtcccgcccctaactccgcccatcccgcccctaactccgcccagttccgcccattctccgccccatggctgactaattttttttatttatgcagaggccgaggccgcctcggcctctgagctattccagaagtagtgaggaggcttttttggaggcctaggcttttgcaaaaagctaacttgtttattgcagcttataatggttacaaataaagcaatagcatcacaaatttcacaaataaagcatttttttcactgcattctagttgtggtttgtccaaactcatcaatgtatcttatcatgtctggatccgctgcattaatgaatcggccaacgcgcggggagaggcggtttgcgtattgggcgctcttccgcttcctcgctcactgactcgctgcgctcggtcgttcggctgcggcgagcggtatcagctcactcaaaggcggtaatacggttatccacagaatcaggggataacgcaggaaagaacatgtgagcaaaaggccagcaaaaggccaggaaccgtaaaaaggccgcgttgctggcgtttttccataggctccgcccccctgacgagcatcacaaaaatcgacgctcaagtcagaggtggcgaaacccgacaggactataaagataccaggcgtttccccctggaagctccctcgtgcgctctcctgttccgaccctgccgcttaccggatacctgtccgcctttctcccttcgggaagcgtggcgctttctcatagctcacgctgtaggtatctcagttcggtgtaggtcgttcgctccaagctgggctgtgtgcacgaaccccccgttcagcccgaccgctgcgccttatccggtaactatcgtcttgagtccaacccggtaagacacgacttatcgccactggcagcagccactggtaacaggattagcagagcgaggtatgtaggcggtgctacagagttcttgaagtggtggcctaactacggctacactagaagaacagtatttggtatctgcgctctgctgaagccagttaccttcggaaaaagagttggtagctcttgatccggcaaacaaaccaccgctggtagcggtggtttttttgtttgcaagcagcagattacgcgcagaaaaaaaggatctcaagaagatcctttgatcttttctacggggtctgacgctcagtggaacgaaaactcacgttaagggattttggtcatgagattatcaaaaaggatcttcacctagatccttttaaattaaaaatgaagttttaaatcaatctaaagtatatatgagtaaacttggtctgacagttaccaatgcttaatcagtgaggcacctatctcagcgatctgtctatttcgttcatccatagttgcctgactccccgtcgtgtagataactacgatacgggagggcttaccatctggccccagtgctgcaatgataccgcgagacccacgctcaccggctccagatttatcagcaataaaccagccagccggaagggccgagcgcagaagtggtcctgcaactttatccgcctccatccagtctattaattgttgccgggaagctagagtaagtagttcgccagttaatagtttgcgcaacgttgttgccattgctacaggcatcgtggtgtcacgctcgtcgtttggtatggcttcattcagctccggttcccaacgatcaaggcgagttacatgatcccccatgttgtgcaaaaaagcggttagctccttcggtcctccgatcgttgtcagaagtaagttggccgcagtgttatcactcatggttatggcagcactgcataattctcttactgtcatgccatccgtaagatgcttttctgtgactggtgagtactcaaccaagtcattctgagaatagtgtatgcggcgaccgagttgctcttgcccggcgtcaatacgggataataccgcgccacatagcagaactttaaaagtgctcatcattggaaaacgttcttcggggcgaaaactctcaaggatcttaccgctgttgagatccagttcgatgtaacccactcgtgcacccaactgatcttcagcatcttttactttcaccagcgtttctgggtgagcaaaaacaggaaggcaaaatgccgcaaaaaagggaataagggcgacacggaaatgttgaatactcatactcttcctttttcaatattattgaagcatttatcagggttattgtctcatgagcggatacatatttgaatgtatttagaaaaataaacaaataggggttccgcgcacatttccccgaaaagtgccacctgg

SEQ ID NO: 6 - DNA, 80 bp, Unknown
  Woodchuck Hepatitis Virus Posttranscriptional Regulatory Element Alpha Component
gccacggcggaactcatcgccgcctgccttgcccgctgctggacaggggctcggctgttgggcactgacaattccgtggt

SEQ ID NO: 7 - DNA, 592 bp, Unknown
  Woodchuck Hepatitis Virus Posttranscriptional Regulatory Element
aatcaacctctggattacaaaatttgtgaaagattgactggtattcttaactatgttgctccttttacgctatgtggatacgctgctttaatgcctttgtatcatgctattgcttcccgtatggctttcattttctcctccttgtataaatcctggttgctgtctctttatgaggagttgtggcccgttgtcaggcaacgtggcgtggtgtgcactgtgtttgctgacgcaacccccactggttggggcattgccaccacctgtcagctcctttccgggactttcgctttccccctccctattgccacggcggaactcatcgccgcctgccttgcccgctgctggacaggggctcggctgttgggcactgacaattccgtggtgttgtcggggaagctgacgtcctttccatggctgctcgcctgtgttgccacctggattctgcgcgggacgtccttctgctacgtcccttcggccctcaatccagcggaccttccttcccgcggcctgctgccggctctgcggcctcttccgcgtcttcgccttcgccctcagacgagtcggatctccctttgggccgcctccccgcctg

SEQ ID NO: 8 - protein, 18 aa, Unknown
  T2A
EGRGSLLTCGDVEENPGP

SEQ ID NO: 9 - protein, 19 aa, Unknown
  P2A
ATNFSLLKQAGDVEENPGP

SEQ ID NO: 10 - protein, 20 aa, Unknown
  E2A
QCTNYALLKLAGDVESNPGP

SEQ ID NO: 11 - protein, 22 aa, Unknown
  F2A
VKQTLNFDLLKLAGDVESNPGP

SEQ ID NO: 12 - protein, 21 aa, Unknown
  T2A
GSGEGRGSLLTCGDVEENPGP

SEQ ID NO: 13 - protein, 22 aa, Unknown
  P2A
GSGATNFSLLKQAGDVEENPGP

SEQ ID NO: 14 - protein, 23 aa, Unknown
  E2A
GSGQCTNYALLKLAGDVESNPGP

SEQ ID NO: 15 - protein, 25 aa, Unknown
  F2A
GSGVKQTLNFDLLKLAGDVESNPGP

SEQ ID NO: 16 - DNA, 11111 bp, Unknown
  64-AAV-CAR-T-Regs
ctgttttaaaagaaaaggggggattggggggtacagtgcaggggaaagaatagtagacataatagcaacagacatacaaactaaagaattacaaaaacaaattacaaaaattcaaaattttatcaacaagcttgatcgatggctccggtgcccgtcagtgggcagagcgcacatcgcccacagtccccgagaagttggggggaggggtcggcaattgaaccggtgcctagagaaggtggcgcggggtaaactgggaaagtgatgtcgtgtactggctccgcctttttcccgagggtgggggagaaccgtatataagtgcagtagtcgccgtgaacgttctttttcgcaacgggtttgccgccagaacacaggtgtcgtgacgcggatccacgcgtgcggccgcacgcgtaagcttagcgcagaggcttggggcagccgagcggcagccaggccccggcccgggcctcggttccagaagggagaggagcccgccaaggcgcgcaagagagcgggctgcctcgcagtccgagccggagagggagcgcgagccgcgccggccccggacggcctcgccgccaccatggctctgcccgtcaccgcactgctgctgcctctggctctgctgctgcacgccgcaagaccagacattgtgctgacacagtctcctgcttccttagctgtatctctggggcagagggccaccatctcatgcagggccagccaaagtgtcagttcatctacctataattttatacactggtatcaacagaaatcaggacagccacccaaactcctcatcaagtatgcatccaacctagaatctggggtccctgtcaggttcagtggcagtgggtctgggacagacttctccctcaacatccatcctgtggaggaggaggatactgcaacatattactgtcagcacagttgggagattccatacacgttcggagggggggccaagttggagataaaaggcagtactagcggtggtggctccgggggcggttccggtgggggcggcagcagccaggtgcagctgaaggagtcaggacctggcctggtggcaccctcacagagcctgtccatcacatgcaccgtctcaggattctcattaagcggctatggcataagctgggttcgccagcctccaggaaagcgtctggaatggctgggattgatatggggtgatggaaccacagactataattcagctctcaaatccagactgagcatcagcaaggacaactccaagagccaggttttcttaaaaatgaacagtctgcaaactgatgacacagccaggtacttctgtaccagagggcctccggccttctataagtacctctactttgactactggggccaaggcaccactctcacagtctcctcactcgaccccaaatcttctgacaaaactcacacatgcccaccgtgcccagcacctcctgtggcaggaccgtcagtcttcctcttccccccaaaacccaaggacaccctcatgatctcccggacccctgaggtcacatgcgtggtggtggacgtgagccacgaagaccctgaggtcaagttcaactggtacgtggacggcgtggaggtgcataatgccaagacaaagccgcgggaggagcagtaccagagcacgtaccgtgtggtcagcgtcctcaccgtcctgcaccaggactggctgaatggcaaggagtacaagtgcaaggtctccaacaaagccctcccagcccccatcgagaaaaccatctccaaagccaaagggcagccccgagaaccacaggtgtacaccctgccaccatcacgagatgagctgaccaagaaccaggtcagcctgacctgcctggtcaaaggcttctatcccagcgacatcgccgtggagtgggagagcaatgggcagccggagaacaactacaagaccacgcctcccgtgctggactccgacggctccttcttcctctacagcaagctcaccgtggacaagagcaggtggcagcaggggaacgtcttctcatgctccgtgatgcatgaggctctgcacaaccactacacgcagaagagcctctccctgtctcccttttgggtgctggtggtggttggtggagtcctggcttgctatagcttgctagtaacagtggcctttattattttctgggtgaggagtaagaggagcaggggaggtcacagtgactacatgaacatgactccccgccgccccgggcccacccgcaagcattaccagccctatgccccaccacgcgacttcgcagcctatcgctccaaacggggcagaaagaaactcctgtatatattcaaacaaccatttatgagaccagtacaaactactcaagaggaagatggctgtagctgccgatttccagaagaagaagaaggaggatgtgaactgagagtgaagttcagcaggagcgcagacgcccccgcgtaccagcagggccagaaccagctctataacgagctcaatctaggacgaagagaggagtacgatgttttggacaagagacgtggccgggaccctgagatggggggaaagccgagaaggaagaaccctcaggaaggcctgtacaatgaactgcagaaagataagatggcggaggcctacagtgagattgggatgaaaggcgagcgccggaggggcaaggggcacgatggcctttaccagggtctcagtacagccaccaaggacacctacgacgcccttcacatgcaggccctgccccctcgccagtgtactaattatgctctcttgaaattggctggagatgttgagagcaaccccgggccggaattcatgcccaaccctaggccagccaagcctatggctccttccttggcccttggcccatccccaggagtcttgccaagctggaagactgcacccaagggctcagaacttctagggaccaggggctctgggggacccttccaaggtcgggacctgcgaagtggggcccacacctcttcttccttgaaccccctgccaccatcccagctgcagctgcctacagtgcccctagtcatggtggcaccgtctggggcccgactaggtccctcaccccacctacaggcccttctccaggacagaccacacttcatgcatcagctctccactgtggatgcccatgcccagacccctgtgctccaagtgcgtccactggacaacccagccatgatcagcctcccaccaccttctgctgccactggggtcttctccctcaaggcccggcctggcctgccacctgggatcaatgtggccagtctggaatgggtgtccagggagccagctctactctgcaccttcccacgctcgggtacacccaggaaagacagcaaccttttggctgcaccccaaggatcctacccactgctggcaaatggagtctgcaagtggcctggttgtgagaaggtcttcgaggagccagaagagtttctcaagcactgccaagcagatcatctcctggatgagaaaggcaaggcccagtgcctcctccagagagaagtggtgcagtctctggagcagcagctggagctggaaaaggagaagctgggagctatgcaggcccacctggctgggaagatggcgctggccaaggctccatctgtggcctcaatggacaagagctcttgctgcatcgtagccaccagtactcagggcagtgtgctcccggcctggtctgctcctcgggaggctccagacggcggcctgtttgcagtgcggaggcacctctggggaagccatggcaatagttccttcccagagttcttccacaacatggactacttcaagtaccacaatatgcgaccccctttcacctatgccacccttatccgatgggccatcctggaagccccggagaggcagaggacactcaatgaaatctaccattggtttactcgcatgttcgcctacttcagaaaccaccccgccacctggaagaatgccatccgccacaacctgagcctgcacaagtgctttgtgcgagtggagagcgagaagggagcagtgtggaccgtagatgaatttgagtttcgcaagaagaggagccaacgccccaacaagtgctccaatccctgcccccagtgtactaattatgctctcttgaaattggctggagatgttgagagcaaccccgggccgatgccacctcctcgcctcctcttcttcctcctcttcctcacccccatggaagtcaggcccgaggaacctctagtggtgaaggtggaagagggagataacgctgtgctgcagtgcctcaaggggacctcagatggccccactcagcagctgacctggtctcgggagtccccgcttaaacccttcttaaaactcagcctggggctgccaggcctgggaatccacatgaggcccctggccatctggcttttcatcttcaacgtctctcaacagatggggggcttctacctgtgccagccggggcccccctctgagaaggcctggcagcctggctggacagtcaatgtggagggcagcggggagctgttccggtggaatgtttcggacctaggtggcctgggctgtggcctgaagaacaggtcctcagagggccccagctccccttccgggaagctcatgagccccaagctgtatgtgtgggccaaagaccgccctgagatctgggagggagagcctccgtgtgtcccaccgagggacagcctgaaccagagcctcagccaggacctcaccatggcccctggctccacactctggctgtcctgtggggtaccccctgactctgtgtccaggggccccctctcctggacccatgtgcaccccaaggggcctaagtcattgctgagcctagagctgaaggacgatcgcccggccagagatatgtgggtaatggagacgggtctgttgttgccccgggccacagctcaagacgctggaaagtattattgtcaccgtggcaacctgaccatgtcattccacctggagatcactgctcggccagtactatggcactggctgctgaggactggtggctggaaggtctcagctgtgactttggcttatctgatcttctgcctgtgttcccttgtgggcattcttcatcttcaaagagccctggtcctgaggaggaaaagatgatctagataaattcgagcatcttaccgccatttattcccatatttgttctgtttttcttgatttgggtatacatttaaatgttaataaaacaaaatggtggggcaatcatttacatttttagggatatgtaattactagttcaggtgtattgccacaagacaaacatgttaagaaactttcccgttatttacgctctgttcctgttaatcaacctctggattacaaaatttgtgaaagattgactgatattcttaactatgttgctccttttacgctgtgtggatatgctgctttatagcctctgtatctagctattgcttcccgtacggctttcgttttctcctccttgtataaatcctggttgctgtctcttttagaggagttgtggcccgttgtccgtcaacgtggcgtggtgtgctctgtgtttgctgacgcaacccccactggctggggcattgccaccacctgtcaactcctttctgggactttcgctttccccctcccgatcgccacggcagaactcatcgccgcctgccttgcccgctgctggacaggggctaggttgctgggcactgataattccgtggtgttgtcggggaagctgacgtcctttcctcgagggggggcccggtacctttaagaccaatgacttacaaggcagctgtagatcttagccactttttaaaagaaaaggggggactggaagggctaattcactcccaacgaagacaagatctgctttttgcttgtactgggtctctctggttagaccagatctgagcctgggagctctctggctaactagggaacccactgcttaagcctcaataaagcttgccttgagtgcttcaagtagtgtgtgcccgtctgttgtgtgactctggtaactagagatccctcagacccttttagtcagtgtggaaaatctctagcagtagtagttcatgtcatcttattattcagtatttataacttgcaaagaaatgaatatcagagagtgagaggaacttgtttattgcagcttataatggttacaaataaagcaatagcatcacaaatttcacaaataaagcatttttttcactgcattctagttgtggtttgtccaaactcatcaatgtatcttatcatgtctggctctagctatcccgcccctaactccgcccagttccgcccattctccgccccatggctgactaattttttttatttatgcagaggccgaggccgcctcggcctctgagctattccagaagtagtgaggaggcttttttggaggcctaggcttttgcgtcgagacgtacccaattcgccctatagtgagtcgtattacgcgcgctcactggccgtcgttttacaacgtcgtgactgggaaaaccctggcgttacccaacttaatcgccttgcagcacatccccctttcgccagctggcgtaatagcgaagaggcccgcaccgatcgcccttcccaacagttgcgcagcctgaatggcgaatggcgcgacgcgccctgtagcggcgcattaagcgcggcgggtgtggtggttacgcgcagcgtgaccgctacacttgccagcgccctagcgcccgctcctttcgctttcttcccttcctttctcgccacgttcgccggctttccccgtcaagctctaaatcgggggctccctttagggttccgatttagtgctttacggcacctcgaccccaaaaaacttgattagggtgatggttcacgtagtgggccatcgccctgatagacggtttttcgccctttgacgttggagtccacgttctttaatagtggactcttgttccaaactggaacaacactcaaccctatctcggtctattcttttgatttataagggattttgccgatttcggcctattggttaaaaaatgagctgatttaacaaaaatttaacgcgaattttaacaaaatattaacgtttacaatttcccaggtggcacttttcggggaaatgtgcgcggaacccctatttgtttatttttctaaatacattcaaatatgtatccgctcatgagacaataaccctgataaatgcttcaataatattgaaaaaggaagagtatgagtattcaacatttccgtgtcgcccttattcccttttttgcggcattttgccttcctgtttttgctcacccagaaacgctggtgaaagtaaaagatgctgaagatcagttgggtgcacgagtgggttacatcgaactggatctcaacagcggtaagatccttgagagttttcgccccgaagaacgttttccaatgatgagcacttttaaagttctgctatgtggcgcggtattatcccgtattgacgccgggcaagagcaactcggtcgccgcatacactattctcagaatgacttggttgagtactcaccagtcacagaaaagcatcttacggatggcatgacagtaagagaattatgcagtgctgccataaccatgagtgataacactgcggccaacttacttctgacaacgatcggaggaccgaaggagctaaccgcttttttgcacaacatgggggatcatgtaactcgccttgatcgttgggaaccggagctgaatgaagccataccaaacgacgagcgtgacaccacgatgcctgtagcaatggcaacaacgttgcgcaaactattaactggcgaactacttactctagcttcccggcaacaattaatagactggatggaggcggataaagttgcaggaccacttctgcgctcggcccttccggctggctggtttattgctgataaatctggagccggtgagcgtgggtctcgcggtatcattgcagcactggggccagatggtaagccctcccgtatcgtagttatctacacgacggggagtcaggcaactatggatgaacgaaatagacagatcgctgagataggtgcctcactgattaagcattggtaactgtcagaccaagtttactcatatatactttagattgatttaaaacttcatttttaatttaaaaggatctaggtgaagatcctttttgataatctcatgaccaaaatcccttaacgtgagttttcgttccactgagcgtcagaccccgtagaaaagatcaaaggatcttcttgagatcctttttttctgcgcgtaatctgctgcttgcaaacaaaaaaaccaccgctaccagcggtggtttgtttgccggatcaagagctaccaactctttttccgaaggtaactggcttcagcagagcgcagataccaaatactgtccttctagtgtagccgtagttaggccaccacttcaagaactctgtagcaccgcctacatacctcgctctgctaatcctgttaccagtggctgctgccagtggcgataagtcgtgtcttaccgggttggactcaagacgatagttaccggataaggcgcagcggtcgggctgaacggggggttcgtgcacacagcccagcttggagcgaacgacctacaccgaactgagatacctacagcgtgagctatgagaaagcgccacgcttcccgaagggagaaaggcggacaggtatccggtaagcggcagggtcggaacaggagagcgcacgagggagcttccagggggaaacgcctggtatctttatagtcctgtcgggtttcgccacctctgacttgagcgtcgatttttgtgatgctcgtcaggggggcggagcctatggaaaaacgccagcaacgcggcctttttacggttcctggccttttgctggccttttgctcacatgttctttcctgcgttatcccctgattctgtggataaccgtattaccgcctttgagtgagctgataccgctcgccgcagccgaacgaccgagcgcagcgagtcagtgagcgaggaagcggaagagcgcccaatacgcaaaccgcctctccccgcgcgttggccgattcattaatgcagctggcacgacaggtttcccgactggaaagcgggcagtgagcgcaacgcaattaatgtgagttagctcactcattaggcaccccaggctttacactttatgcttccggctcgtatgttgtgtggaattgtgagcggataacaatttcacacaggaaacagctatgaccatgattacgccaagcgcgcaattaaccctcactaaagggaacaaaagctggagctgcaagcttaatgtagtcttatgcaatactcttgtagtcttgcaacatggtaacgatgagttagcaacatgccttacaaggagagaaaaagcaccgtgcatgccgattggtggaagtaaggtggtacgatcgtgccttattaggaaggcaacagacgggtctgacatggattggacgaaccactgaattgccgcattgcagagatattgtatttaagtgcctagctcgatacataaacgggtctctctggttagaccagatctgagcctgggagctctctggctaactagggaacccactgcttaagcctcaataaagcttgccttgagtgcttcaagtagtgtgtgcccgtctgttgtgtgactctggtaactagagatccctcagacccttttagtcagtgtggaaaatctctagcagtggcgcccgaacagggacttgaaagcgaaagggaaaccagaggagctctctcgacgcaggactcggcttgctgaagcgcgcacggcaagaggcgaggggcggcgactggtgagtacgccaaaaattttgactagcggaggctagaaggagagagatgggtgcgagagcgtcagtattaagcgggggagaattagatcgcgatgggaaaaaattcggttaaggccagggggaaagaaaaaatataaattaaaacatatagtatgggcaagcagggagctagaacgattcgcagttaatcctggcctgttagaaacatcagaaggctgtagacaaatactgggacagctacaaccatcccttcagacaggatcagaagaacttagatcattatataatacagtagcaaccctctattgtgtgcatcaaaggatagagataaaagacaccaaggaagctttagacaagatagaggaagagcaaaacaaaagtaagaccaccgcacagcaagcggccgctgatcttcagacctggaggaggagatatgagggacaattggagaagtgaattatataaatataaagtagtaaaaattgaaccattaggagtagcacccaccaaggcaaagagaagagtggtgcagagagaaaaaagagcagtgggaataggagctttgttccttgggttcttgggagcagcaggaagcactatgggcgcagcctcaatgacgctgacggtacaggccagacaattattgtctggtatagtgcagcagcagaacaatttgctgagggctattgaggcgcaacagcatctgttgcaactcacagtctggggcatcaagcagctccaggcaagaatcctggctgtggaaagatacctaaaggatcaacagctcctggggatttggggttgctctggaaaactcatttgcaccactgctgtgccttggaatgctagttggagtaataaatctctggaacagatttggaatcacacgacctggatggagtgggacagagaaattaacaattacacaagcttaatacactccttaattgaagaatcgcaaaaccagcaagaaaagaatgaacaagaattattggaattagataaatgggcaagtttgtggaattggtttaacataacaaattggctgtggtatataaaattattcataatgatagtaggaggcttggtaggtttaagaatagtttttgctgtactttctatagtgaatagagttaggcagggatattcaccattatcgtttcagacccacctcccaaccccgaggggacccgacaggcccgaaggaatagaagaagaaggtggagagagagacagagacagatccattcgattagtgaacggatctcgacggtatcggtt

SEQ ID NO: 17 - DNA, 9764 bp, Unknown
  65-AAV-CAR-T-Cells
ctgttttaaaagaaaaggggggattggggggtacagtgcaggggaaagaatagtagacataatagcaacagacatacaaactaaagaattacaaaaacaaattacaaaaattcaaaattttatcaacaagcttgatcgatggctccggtgcccgtcagtgggcagagcgcacatcgcccacagtccccgagaagttggggggaggggtcggcaattgaaccggtgcctagagaaggtggcgcggggtaaactgggaaagtgatgtcgtgtactggctccgcctttttcccgagggtgggggagaaccgtatataagtgcagtagtcgccgtgaacgttctttttcgcaacgggtttgccgccagaacacaggtgtcgtgacgcggatccacgcgtgcggccgcacgcgtaagcttagcgcagaggcttggggcagccgagcggcagccaggccccggcccgggcctcggttccagaagggagaggagcccgccaaggcgcgcaagagagcgggctgcctcgcagtccgagccggagagggagcgcgagccgcgccggccccggacggcctcgccgccaccatggctctgcccgtcaccgcactgctgctgcctctggctctgctgctgcacgccgcaagaccagacattgtgctgacacagtctcctgcttccttagctgtatctctggggcagagggccaccatctcatgcagggccagccaaagtgtcagttcatctacctataattttatacactggtatcaacagaaatcaggacagccacccaaactcctcatcaagtatgcatccaacctagaatctggggtccctgtcaggttcagtggcagtgggtctgggacagacttctccctcaacatccatcctgtggaggaggaggatactgcaacatattactgtcagcacagttgggagattccatacacgttcggagggggggccaagttggagataaaaggcagtactagcggtggtggctccgggggcggttccggtgggggcggcagcagccaggtgcagctgaaggagtcaggacctggcctggtggcaccctcacagagcctgtccatcacatgcaccgtctcaggattctcattaagcggctatggcataagctgggttcgccagcctccaggaaagcgtctggaatggctgggattgatatggggtgatggaaccacagactataattcagctctcaaatccagactgagcatcagcaaggacaactccaagagccaggttttcttaaaaatgaacagtctgcaaactgatgacacagccaggtacttctgtaccagagggcctccggccttctataagtacctctactttgactactggggccaaggcaccactctcacagtctcctcactcgaccccaaatcttctgacaaaactcacacatgcccaccgtgcccagcacctcctgtggcaggaccgtcagtcttcctcttccccccaaaacccaaggacaccctcatgatctcccggacccctgaggtcacatgcgtggtggtggacgtgagccacgaagaccctgaggtcaagttcaactggtacgtggacggcgtggaggtgcataatgccaagacaaagccgcgggaggagcagtaccagagcacgtaccgtgtggtcagcgtcctcaccgtcctgcaccaggactggctgaatggcaaggagtacaagtgcaaggtctccaacaaagccctcccagcccccatcgagaaaaccatctccaaagccaaagggcagccccgagaaccacaggtgtacaccctgccaccatcacgagatgagctgaccaagaaccaggtcagcctgacctgcctggtcaaaggcttctatcccagcgacatcgccgtggagtgggagagcaatgggcagccggagaacaactacaagaccacgcctcccgtgctggactccgacggctccttcttcctctacagcaagctcaccgtggacaagagcaggtggcagcaggggaacgtcttctcatgctccgtgatgcatgaggctctgcacaaccactacacgcagaagagcctctccctgtctcccttttgggtgctggtggtggttggtggagtcctggcttgctatagcttgctagtaacagtggcctttattattttctgggtgaggagtaagaggagcaggggaggtcacagtgactacatgaacatgactccccgccgccccgggcccacccgcaagcattaccagccctatgccccaccacgcgacttcgcagcctatcgctccaaacggggcagaaagaaactcctgtatatattcaaacaaccatttatgagaccagtacaaactactcaagaggaagatggctgtagctgccgatttccagaagaagaagaaggaggatgtgaactgagagtgaagttcagcaggagcgcagacgcccccgcgtaccagcagggccagaaccagctctataacgagctcaatctaggacgaagagaggagtacgatgttttggacaagagacgtggccgggaccctgagatggggggaaagccgagaaggaagaaccctcaggaaggcctgtacaatgaactgcagaaagataagatggcggaggcctacagtgagattgggatgaaaggcgagcgccggaggggcaaggggcacgatggcctttaccagggtctcagtacagccaccaaggacacctacgacgcccttcacatgcaggccctgccccctcgccagtgtactaattatgctctcttgaaattggctggagatgttgagagcaaccccgggccggaattcatgccacctcctcgcctcctcttcttcctcctcttcctcacccccatggaagtcaggcccgaggaacctctagtggtgaaggtggaagagggagataacgctgtgctgcagtgcctcaaggggacctcagatggccccactcagcagctgacctggtctcgggagtccccgcttaaacccttcttaaaactcagcctggggctgccaggcctgggaatccacatgaggcccctggccatctggcttttcatcttcaacgtctctcaacagatggggggcttctacctgtgccagccggggcccccctctgagaaggcctggcagcctggctggacagtcaatgtggagggcagcggggagctgttccggtggaatgtttcggacctaggtggcctgggctgtggcctgaagaacaggtcctcagagggccccagctccccttccgggaagctcatgagccccaagctgtatgtgtgggccaaagaccgccctgagatctgggagggagagcctccgtgtgtcccaccgagggacagcctgaaccagagcctcagccaggacctcaccatggcccctggctccacactctggctgtcctgtggggtaccccctgactctgtgtccaggggccccctctcctggacccatgtgcaccccaaggggcctaagtcattgctgagcctagagctgaaggacgatcgcccggccagagatatgtgggtaatggagacgggtctgttgttgccccgggccacagctcaagacgctggaaagtattattgtcaccgtggcaacctgaccatgtcattccacctggagatcactgctcggccagtactatggcactggctgctgaggactggtggctggaaggtctcagctgtgactttggcttatctgatcttctgcctgtgttcccttgtgggcattcttcatcttcaaagagccctggtcctgaggaggaaaagatgatctagataaattcgagcatcttaccgccatttattcccatatttgttctgtttttcttgatttgggtatacatttaaatgttaataaaacaaaatggtggggcaatcatttacatttttagggatatgtaattactagttcaggtgtattgccacaagacaaacatgttaagaaactttcccgttatttacgctctgttcctgttaatcaacctctggattacaaaatttgtgaaagattgactgatattcttaactatgttgctccttttacgctgtgtggatatgctgctttatagcctctgtatctagctattgcttcccgtacggctttcgttttctcctccttgtataaatcctggttgctgtctcttttagaggagttgtggcccgttgtccgtcaacgtggcgtggtgtgctctgtgtttgctgacgcaacccccactggctggggcattgccaccacctgtcaactcctttctgggactttcgctttccccctcccgatcgccacggcagaactcatcgccgcctgccttgcccgctgctggacaggggctaggttgctgggcactgataattccgtggtgttgtcggggaagctgacgtcctttcctcgagggggggcccggtacctttaagaccaatgacttacaaggcagctgtagatcttagccactttttaaaagaaaaggggggactggaagggctaattcactcccaacgaagacaagatctgctttttgcttgtactgggtctctctggttagaccagatctgagcctgggagctctctggctaactagggaacccactgcttaagcctcaataaagcttgccttgagtgcttcaagtagtgtgtgcccgtctgttgtgtgactctggtaactagagatccctcagacccttttagtcagtgtggaaaatctctagcagtagtagttcatgtcatcttattattcagtatttataacttgcaaagaaatgaatatcagagagtgagaggaacttgtttattgcagcttataatggttacaaataaagcaatagcatcacaaatttcacaaataaagcatttttttcactgcattctagttgtggtttgtccaaactcatcaatgtatcttatcatgtctggctctagctatcccgcccctaactccgcccagttccgcccattctccgccccatggctgactaattttttttatttatgcagaggccgaggccgcctcggcctctgagctattccagaagtagtgaggaggcttttttggaggcctaggcttttgcgtcgagacgtacccaattcgccctatagtgagtcgtattacgcgcgctcactggccgtcgttttacaacgtcgtgactgggaaaaccctggcgttacccaacttaatcgccttgcagcacatccccctttcgccagctggcgtaatagcgaagaggcccgcaccgatcgcccttcccaacagttgcgcagcctgaatggcgaatggcgcgacgcgccctgtagcggcgcattaagcgcggcgggtgtggtggttacgcgcagcgtgaccgctacacttgccagcgccctagcgcccgctcctttcgctttcttcccttcctttctcgccacgttcgccggctttccccgtcaagctctaaatcgggggctccctttagggttccgatttagtgctttacggcacctcgaccccaaaaaacttgattagggtgatggttcacgtagtgggccatcgccctgatagacggtttttcgccctttgacgttggagtccacgttctttaatagtggactcttgttccaaactggaacaacactcaaccctatctcggtctattcttttgatttataagggattttgccgatttcggcctattggttaaaaaatgagctgatttaacaaaaatttaacgcgaattttaacaaaatattaacgtttacaatttcccaggtggcacttttcggggaaatgtgcgcggaacccctatttgtttatttttctaaatacattcaaatatgtatccgctcatgagacaataaccctgataaatgcttcaataatattgaaaaaggaagagtatgagtattcaacatttccgtgtcgcccttattcccttttttgcggcattttgccttcctgtttttgctcacccagaaacgctggtgaaagtaaaagatgctgaagatcagttgggtgcacgagtgggttacatcgaactggatctcaacagcggtaagatccttgagagttttcgccccgaagaacgttttccaatgatgagcacttttaaagttctgctatgtggcgcggtattatcccgtattgacgccgggcaagagcaactcggtcgccgcatacactattctcagaatgacttggttgagtactcaccagtcacagaaaagcatcttacggatggcatgacagtaagagaattatgcagtgctgccataaccatgagtgataacactgcggccaacttacttctgacaacgatcggaggaccgaaggagctaaccgcttttttgcacaacatgggggatcatgtaactcgccttgatcgttgggaaccggagctgaatgaagccataccaaacgacgagcgtgacaccacgatgcctgtagcaatggcaacaacgttgcgcaaactattaactggcgaactacttactctagcttcccggcaacaattaatagactggatggaggcggataaagttgcaggaccacttctgcgctcggcccttccggctggctggtttattgctgataaatctggagccggtgagcgtgggtctcgcggtatcattgcagcactggggccagatggtaagccctcccgtatcgtagttatctacacgacggggagtcaggcaactatggatgaacgaaatagacagatcgctgagataggtgcctcactgattaagcattggtaactgtcagaccaagtttactcatatatactttagattgatttaaaacttcatttttaatttaaaaggatctaggtgaagatcctttttgataatctcatgaccaaaatcccttaacgtgagttttcgttccactgagcgtcagaccccgtagaaaagatcaaaggatcttcttgagatcctttttttctgcgcgtaatctgctgcttgcaaacaaaaaaaccaccgctaccagcggtggtttgtttgccggatcaagagctaccaactctttttccgaaggtaactggcttcagcagagcgcagataccaaatactgtccttctagtgtagccgtagttaggccaccacttcaagaactctgtagcaccgcctacatacctcgctctgctaatcctgttaccagtggctgctgccagtggcgataagtcgtgtcttaccgggttggactcaagacgatagttaccggataaggcgcagcggtcgggctgaacggggggttcgtgcacacagcccagcttggagcgaacgacctacaccgaactgagatacctacagcgtgagctatgagaaagcgccacgcttcccgaagggagaaaggcggacaggtatccggtaagcggcagggtcggaacaggagagcgcacgagggagcttccagggggaaacgcctggtatctttatagtcctgtcgggtttcgccacctctgacttgagcgtcgatttttgtgatgctcgtcaggggggcggagcctatggaaaaacgccagcaacgcggcctttttacggttcctggccttttgctggccttttgctcacatgttctttcctgcgttatcccctgattctgtggataaccgtattaccgcctttgagtgagctgataccgctcgccgcagccgaacgaccgagcgcagcgagtcagtgagcgaggaagcggaagagcgcccaatacgcaaaccgcctctccccgcgcgttggccgattcattaatgcagctggcacgacaggtttcccgactggaaagcgggcagtgagcgcaacgcaattaatgtgagttagctcactcattaggcaccccaggctttacactttatgcttccggctcgtatgttgtgtggaattgtgagcggataacaatttcacacaggaaacagctatgaccatgattacgccaagcgcgcaattaaccctcactaaagggaacaaaagctggagctgcaagcttaatgtagtcttatgcaatactcttgtagtcttgcaacatggtaacgatgagttagcaacatgccttacaaggagagaaaaagcaccgtgcatgccgattggtggaagtaaggtggtacgatcgtgccttattaggaaggcaacagacgggtctgacatggattggacgaaccactgaattgccgcattgcagagatattgtatttaagtgcctagctcgatacataaacgggtctctctggttagaccagatctgagcctgggagctctctggctaactagggaacccactgcttaagcctcaataaagcttgccttgagtgcttcaagtagtgtgtgcccgtctgttgtgtgactctggtaactagagatccctcagacccttttagtcagtgtggaaaatctctagcagtggcgcccgaacagggacttgaaagcgaaagggaaaccagaggagctctctcgacgcaggactcggcttgctgaagcgcgcacggcaagaggcgaggggcggcgactggtgagtacgccaaaaattttgactagcggaggctagaaggagagagatgggtgcgagagcgtcagtattaagcgggggagaattagatcgcgatgggaaaaaattcggttaaggccagggggaaagaaaaaatataaattaaaacatatagtatgggcaagcagggagctagaacgattcgcagttaatcctggcctgttagaaacatcagaaggctgtagacaaatactgggacagctacaaccatcccttcagacaggatcagaagaacttagatcattatataatacagtagcaaccctctattgtgtgcatcaaaggatagagataaaagacaccaaggaagctttagacaagatagaggaagagcaaaacaaaagtaagaccaccgcacagcaagcggccgctgatcttcagacctggaggaggagatatgagggacaattggagaagtgaattatataaatataaagtagtaaaaattgaaccattaggagtagcacccaccaaggcaaagagaagagtggtgcagagagaaaaaagagcagtgggaataggagctttgttccttgggttcttgggagcagcaggaagcactatgggcgcagcctcaatgacgctgacggtacaggccagacaattattgtctggtatagtgcagcagcagaacaatttgctgagggctattgaggcgcaacagcatctgttgcaactcacagtctggggcatcaagcagctccaggcaagaatcctggctgtggaaagatacctaaaggatcaacagctcctggggatttggggttgctctggaaaactcatttgcaccactgctgtgccttggaatgctagttggagtaataaatctctggaacagatttggaatcacacgacctggatggagtgggacagagaaattaacaattacacaagcttaatacactccttaattgaagaatcgcaaaaccagcaagaaaagaatgaacaagaattattggaattagataaatgggcaagtttgtggaattggtttaacataacaaattggctgtggtatataaaattattcataatgatagtaggaggcttggtaggtttaagaatagtttttgctgtactttctatagtgaatagagttaggcagggatattcaccattatcgtttcagacccacctcccaaccccgaggggacccgacaggcccgaaggaatagaagaagaaggtggagagagagacagagacagatccattcgattagtgaacggatctcgacggtatcggtt

SEQ ID NO: 18 - DNA, 291 bp, Unknown
  EF1-alpha
aacaagcttgatcgatggctccggtgcccgtcagtgggcagagcgcacatcgcccacagtccccgagaagttggggggaggggtcggcaattgaaccggtgcctagagaaggtggcgcggggtaaactgggaaagtgatgtcgtgtactggctccgcctttttcccgagggtgggggagaaccgtatataagtgcagtagtcgccgtgaacgttctttttcgcaacgggtttgccgccagaacacaggtgtcgtgacgcggatccacgcgtgcggccgcacgcgtaagctt

SEQ ID NO: 19 - DNA, 584 bp, Unknown
  CMV
ggcattgattattgactagttattaatagtaatcaattacggggtcattagttcatagcccatatatggagttccgcgttacataacttacggtaaatggcccgcctggctgaccgcccaacgacccccgcccattgacgtcaataatgacgtatgttcccatagtaacgccaatagggactttccattgacgtcaatgggtggagtatttacggtaaactgcccacttggcagtacatcaagtgtatcatatgccaagtccgccccctattgacgtcaatgacggtaaatggcccgcctggcattatgcccagtacatgaccttacgggactttcctacttggcagtacatctacgtattagtcatcgctattaccatggtgatgcggttttggcagtacaccaatgggcgtggatagcggtttgactcacggggatttccaagtctccaccccattgacgtcaatgggagtttgttttggcaccaaaatcaacgggactttccaaaatgtcgtaataaccccgccccgttgacgcaaatgggcggtaggcgtgtacggtgggaggtctatataagcagaggt

SEQ ID NO: 20 - DNA, 450 bp, Unknown
  MND2
ggccgccagtgtgatggatatctgcagaattcgcccttatggggatccgaacagagagacagcagaatatgggccaaacaggatatctgtggtaagcagttcctgccccggctcagggccaagaacagttggaacagcagaatatgggccaaacaggatatctgtggtaagcagttcctgccccggctcagggccaagaacagatggtccccagatgcggtcccgccctcagcagtttctagagaaccatcagatgtttccagggtgccccaaggacctgaaatgaccctgtgccttatttgaactaaccaatcagttcgcttctcgcttctgttcgcgcgcttctgctccccgagctctatataagcagagctcgtttagtgaaccgtcagatcgcctggagacgccatccacgctgttttgacctccatagaagacaccgactctaga

SEQ ID NO: 21 - DNA, 408 bp, Unknown
  SFFV
gtaacgccattttgcaaggcatggaaaaataccaaaccaagaatagagaagttcagatcaagggcgggtacatgaaaatagctaacgttgggccaaacaggatatctgcggtgagcagtttcggccccggcccggggccaagaacagatggtcaccgcagtttcggccccggcccgaggccaagaacagatggtccccagatatggcccaaccctcagcagtttcttaagacccatcagatgtttccaggctcccccaaggacctgaaatgaccctgcgccttatttgaattaaccaatcagcctgcttctcgcttctgttcgcgcgcttctgcttcccgagctctataaaagagctcacaacccctcactcggcgcgccagtcctccgacagactgagtcgcccggg

SEQ ID NO: 22 - DNA, 750 bp, Unknown
  AAV-ScFv
gacattgtgctgacacagtctcctgcttccttagctgtatctctggggcagagggccaccatctcatgcagggccagccaaagtgtcagttcatctacctataattttatacactggtatcaacagaaatcaggacagccacccaaactcctcatcaagtatgcatccaacctagaatctggggtccctgtcaggttcagtggcagtgggtctgggacagacttctccctcaacatccatcctgtggaggaggaggatactgcaacatattactgtcagcacagttgggagattccatacacgttcggagggggggccaagttggagataaaaggcagtactagcggtggtggctccgggggcggttccggtgggggcggcagcagccaggtgcagctgaaggagtcaggacctggcctggtggcaccctcacagagcctgtccatcacatgcaccgtctcaggattctcattaagcggctatggcataagctgggttcgccagcctccaggaaagcgtctggaatggctgggattgatatggggtgatggaaccacagactataattcagctctcaaatccagactgagcatcagcaaggacaactccaagagccaggttttcttaaaaatgaacagtctgcaaactgatgacacagccaggtacttctgtaccagagggcctccggccttctataagtacctctactttgactactggggccaaggcaccactctcacagtctcctca

SEQ ID NO: 23 - DNA, 672 bp, Unknown
  IgG1 hinge-IgG2 hinge, IgG1 CH2CH3
gacaaaactcacacatgcccaccgtgcccagcacctcctgtggcaggaccgtcagtcttcctcttccccccaaaacccaaggacaccctcatgatctcccggacccctgaggtcacatgcgtggtggtggacgtgagccacgaagaccctgaggtcaagttcaactggtacgtggacggcgtggaggtgcataatgccaagacaaagccgcgggaggagcagtaccagagcacgtaccgtgtggtcagcgtcctcaccgtcctgcaccaggactggctgaatggcaaggagtacaagtgcaaggtctccaacaaagccctcccagcccccatcgagaaaaccatctccaaagccaaagggcagccccgagaaccacaggtgtacaccctgccaccatcacgagatgagctgaccaagaaccaggtcagcctgacctgcctggtcaaaggcttctatcccagcgacatcgccgtggagtgggagagcaatgggcagccggagaacaactacaagaccacgcctcccgtgctggactccgacggctccttcttcctctacagcaagctcaccgtggacaagagcaggtggcagcaggggaacgtcttctcatgctccgtgatgcatgaggctctgcacaaccactacacgcagaagagcctctccctgtctccc

SEQ ID NO: 24 - DNA, 117 bp, Unknown
  CD28 extracellular domain
attgaagttatgtatcctcctccttacctagacaatgagaagagcaatggaaccattatccatgtgaaagggaaacacctttgtccaagtcccctatttcccggaccttctaagccc

SEQ ID NO: 25 - DNA, 81 bp, Unknown
  CD28 transmembrane domain
ttttgggtgctggtggtggttggtggagtcctggcttgctatagcttgctagtaacagtggcctttattattttctgggtg

SEQ ID NO: 26 - DNA, 123 bp, Unknown
  Human CD28 signaling domain
aggagtaagaggagcaggggaggtcacagtgactacatgaacatgactccccgccgccccgggcccacccgcaagcattaccagccctatgccccaccacgcgacttcgcagcctatcgctcc

SEQ ID NO: 27 - DNA, 123 bp, Unknown
  Murine CD28 signaling domain
aacagcagaagaaacagaggcggccagagcgactacatgaacatgacccccagaaggccaggcctgaccagaaagccctaccagccctacgcccctgccagagacttcgccgcctacagaccc

SEQ ID NO: 28 - DNA, 126 bp, Unknown
  Human 4-1BB signaling domain
aaacggggcagaaagaaactcctgtatatattcaaacaaccatttatgagaccagtacaaactactcaagaggaagatggctgtagctgccgatttccagaagaagaagaaggaggatgtgaactg

SEQ ID NO: 29 - DNA, 144 bp, Unknown
  Murine 4-1BB signaling domain
tctgtgctcaaatggatcaggaaaaaattcccccacatattcaagcaaccatttaagaagaccactggagcagctcaagaggaagatgcttgtagctgccgatgtccacaggaagaagaaggaggaggaggaggctatgagctg

SEQ ID NO: 30 - DNA, 336 bp, Unknown
  Human CD3z
agagtgaagttcagcaggagcgcagacgcccccgcgtaccagcagggccagaaccagctctataacgagctcaatctaggacgaagagaggagtacgatgttttggacaagagacgtggccgggaccctgagatggggggaaagccgagaaggaagaaccctcaggaaggcctgtacaatgaactgcagaaagataagatggcggaggcctacagtgagattgggatgaaaggcgagcgccggaggggcaaggggcacgatggcctttaccagggtctcagtacagccaccaaggacacctacgacgcccttcacatgcaggccctgccccctcgc

SEQ ID NO: 31 - DNA, 342 bp, Unknown
  Murine CD3z
agagccaagttcagcagatccgccgagacagccgccaacctgcaggatcccaaccagctgtacaacgagctgaacctgggcagacgggaggaatacgacgtgctggaaaagaagagagccagggaccccgagatgggcggcaagcagcagagaagaagaaaccctcaggaaggcgtctacaacgccctgcagaaagacaagatggccgaggcctacagcgagatcggcaccaagggcgagagaagaaggggcaagggccacgatggcctgtaccagggcctgtccaccgccaccaaggacacctacgacgccctgcacatgcagaccctggcccccagatga

SEQ ID NO: 32 - DNA, 969 bp, Unknown
  CD19 extracellular domain
atgccacctcctcgcctcctcttcttcctcctcttcctcacccccatggaagtcaggcccgaggaacctctagtggtgaaggtggaagagggagataacgctgtgctgcagtgcctcaaggggacctcagatggccccactcagcagctgacctggtctcgggagtccccgcttaaacccttcttaaaactcagcctggggctgccaggcctgggaatccacatgaggcccctggccatctggcttttcatcttcaacgtctctcaacagatggggggcttctacctgtgccagccggggcccccctctgagaaggcctggcagcctggctggacagtcaatgtggagggcagcggggagctgttccggtggaatgtttcggacctaggtggcctgggctgtggcctgaagaacaggtcctcagagggccccagctccccttccgggaagctcatgagccccaagctgtatgtgtgggccaaagaccgccctgagatctgggagggagagcctccgtgtgtcccaccgagggacagcctgaaccagagcctcagccaggacctcaccatggcccctggctccacactctggctgtcctgtggggtaccccctgactctgtgtccaggggccccctctcctggacccatgtgcaccccaaggggcctaagtcattgctgagcctagagctgaaggacgatcgcccggccagagatatgtgggtaatggagacgggtctgttgttgccccgggccacagctcaagacgctggaaagtattattgtcaccgtggcaacctgaccatgtcattccacctggagatcactgctcggccagtactatggcactggctgctgaggactggtggctggaaggtctcagctgtgactttggcttatctgatcttctgcctgtgttcccttgtgggcattcttcatcttcaaagagccctggtcctgaggaggaaaaga

SEQ ID NO: 33 - DNA, 1021 bp, Unknown
  EGFR extracellular domain
atgcttctcctggtgacaagccttctgctctgtgagttaccacacccagcattcctcctgatcccacgcaaagtgtgtaacggaataggtattggtgaatttaaagactcactctccataaatgctacgaatattaaacacttcaaaaactgcacctccatcagtggcgatctccacatcctgccggtggcatttaggggtgactccttcacacatactcctcctctggatccacaggaactggatattctgaaaaccgtaaaggaaatcacagggtttttgctgattcaggcttggcctgaaaacaggacggacctccatgcctttgagaacctagaaatcatacgcggcaggaccaagcaacatggtcagttttctcttgcagtcgtcagcctgaacataacatccttgggattacgctccctcaaggagataagtgatggagatgtgataatttcaggaaacaaaaatttgtgctatgcaaatacaataaactggaaaaaactgtttgggacctccggtcagaaaaccaaaattataagcaacagaggtgaaaacagctgcaaggccacaggccaggtctgccatgccttgtgctcccccgagggctgctggggcccggagcccagggactgcgtctcttgccggaatgtcagccgaggcagggaatgcgtggacaagtgcaaccttctggagggtgagccaagggagtttgtggagaactctgagtgcatacagtgccacccagagtgcctgcctcaggccatgaacatcacctgcacaggacggggaccagacaactgtatccagtgtgcccactacattgacggcccccactgcgtcaagacctgcccggcaggagtcatgggagaaaacaacaccctggtctggaagtacgcagacgccggccatgtgtgccacctgtgccatccaaactgcacctacggatgcactgggccaggtcttgaaggctgtccaacgaatgggcctaagatcccgtccatcgccactggatctagat

SEQ ID NO: 34 - DNA, 60 bp, Unknown
  E2A
cagtgtactaattatgctctcttgaaattggctggagatgttgagagcaaccccgggccg

SEQ ID NO: 35 - DNA, 54 bp, Unknown
  T2A
gaaggtcgtggatcactacttacgtgcggtgatgtagaagagaatccgggtccg

SEQ ID NO: 36 - DNA, 57 bp, Unknown
  P2A
gccacaaacttctctctgctaaagcaagcaggtgatgttgaagaaaaccccgggcct

SEQ ID NO: 37 - DNA, 2214 bp, Unknown
  AAV8-capsid
atggctgccgatggttatcttccagattggctcgaggacaacctctctgagggcattcgcgagtggtgggcgctgaaacctggagccccgaagcccaaagccaaccagcaaaagcaggacgacggccggggtctggtgcttcctggctacaagtacctcggacccttcaacggactcgacaagggggagcccgtcaacgcggcggacgcagcggccctcgagcacgacaaggcctacgaccagcagctgcaggcgggtgacaatccgtacctgcggtataaccacgccgacgccgagtttcaggagcgtctgcaagaagatacgtcttttgggggcaacctcgggcgagcagtcttccaggccaagaagcgggttctcgaacctctcggtctggttgaggaaggcgctaagacggctcctggaaagaagagaccggtagagccatcaccccagcgttctccagactcctctacgggcatcggcaagaaaggccaacagcccgccagaaaaagactcaattttggtcagactggcgactcagagtcagttccagaccctcaacctctcggagaacctccagcagcgccctctggtgtgggacctaatacaatggctgcaggcggtggcgcaccaatggcagacaataacgaaggcgccgacggagtgggtagttcctcgggaaattggcattgcgattccacatggctgggcgacagagtcatcaccaccagcacccgaacctgggccctgcccacctacaacaaccacctctacaagcaaatctccaacgggacatcgggaggagccaccaacgacaacacctacttcggctacagcaccccctgggggtattttgactttaacagattccactgccacttttcaccacgtgactggcagcgactcatcaacaacaactggggattccggcccaagagactcagcttcaagctcttcaacatccaggtcaaggaggtcacgcagaatgaaggcaccaagaccatcgccaataacctcaccagcaccatccaggtgtttacggactcggagtaccagctgccgtacgttctcggctctgcccaccagggctgcctgcctccgttcccggcggacgtgttcatgattccccagtacggctacctaacactcaacaacggtagtcaggccgtgggacgctcctccttctactgcctggaatactttccttcgcagatgctgagaaccggcaacaacttccagtttacttacaccttcgaggacgtgcctttccacagcagctacgcccacagccagagcttggaccggctgatgaatcctctgattgaccagtacctgtactacttgtctcggactcaaacaacaggaggcacggcaaatacgcagactctgggcttcagccaaggtgggcctaatacaatggccaatcaggcaaagaactggctgccaggaccctgttaccgccaacaacgcgtctcaacgacaaccgggcaaaacaacaatagcaactttgcctggactgctgggaccaaataccatctgaatggaagaaattcattggctaatcctggcatcgctatggcaacacacaaagacgacgaggagcgtttttttcccagtaacgggatcctgatttttggcaaacaaaatgctgccagagacaatgcggattacagcgatgtcatgctcaccagcgaggaagaaatcaaaaccactaaccctgtggctacagaggaatacggtatcgtggcagataacttgcagcagcaaaacacggctcctcaaattggaactgtcaacagccagggggccttacccggtatggtctggcagaaccgggacgtgtacctgcagggtcccatctgggccaagattcctcacacggacggcaacttccacccgtctccgctgatgggcggctttggcctgaaacatcctccgcctcagatcctgatcaagaacacgcctgtacctgcggatcctccgaccaccttcaaccagtcaaagctgaactctttcatcacgcaatacagcaccggacaggtcagcgtggaaattgaatgggagctgcagaaggaaaacagcaagcgctggaaccccgagatccagtacacctccaactactacaaatctacaagtgtggactttgctgttaatacagaaggcgtgtactctgaaccccgccccattggcacccgttacctcacccgtaatctg

SEQ ID NO: 38 - DNA, 2080 bp, Unknown
  AAV9-capsid
atggctgccgatggttatcttccagattggctcgaggacaaccttagtgaaggaattcgcgagtggtgggctttgaaacctggagcccctcaacccaaggcaaatcaacaacatcaagacaacgctcgaggtcttgtgcttccgggttacaaataccttggacccggcaacggactcgacaagggggagccggtcaacgcagcagacgcggcggccctcgagcacgacaaggcctacgaccagcagctcaaggccggagacaacccgtacctcaagtacaaccacgccgacgccgagttccaggagcggctcaaagaagatacgtcttttgggggcaacctcgggcgagcagtcttccaggccaaaaagaggcttcttgaacctcttggtctggttgaggaagcggctaagacggctcctggaaagaagaggcctgtagagcagtctcctcaggaaccggactcctccgcgggtattggcaaatcgggtgcacagcccgctaaaaagagactcaatttcggtcagactggcgacacagagtcagtcccagaccctcaaccaatcggagaacctcccgcagccccctcaggtgtgggatctcttacaatggcttcaggtggtggcgcaccagtggcagacaataacgaaggtgccgatggagtgggtagttcctcgggaaattggcattgcgattcccaatggctgggggacagagtcatcaccaccagcacccgaacctgggccctgcccacctacaacaatcacctctacaagcaaatctccaacagcacatctggaggatcttcaaatgacaacgcctacttcggctacagcaccccctgggggtattttgacttcaacagattccactgccacttctcaccacgtgactggcagcgactcatcaacaacaactggggattccggcctaagcgactcaacttcaagctcttcaacattcaggtcaaagaggttacggacaacaatggagtcaagaccatcgccaataaccttaccagcacggtccaggtcttcacggactcagactatcagctcccgtacgtgctcgggtcggctcacgagggctgcctcccgccgttcccagcggacgttttcatgattcctcagtacgggtatctgacgcttaatgatggaagccaggccgtgggtcgttcgtccttttactgcctggaatatttcccgtcgcaaatgctaagaacgggtaacaacttccagttcagctacgagtttgagaacgtacctttccatagcagctacgctcacagccaaagcctggaccgactaatgaatccactcatcgaccaatacttgtactatctctcaaagactattaacggttctggacagaatcaacaaacgctaaaattcagtgtggccggacccagcaacatggctgtccagggaagaaactacatacctggacccagctaccgacaacaacgtgtctcaaccactgtgactcaaaacaacaacagcgaatttgcttggcctggagcttcttcttgggctctcaatggacgtaatagcttgatgaatcctggacctgctatggccagccacaaagaaggagaggaccgtttctttcctttgtctggatctttaatttttggcaaacaaggaactggaagagacaacgtggatgcggacaaagtcatgataaccaacgaagaagaaattaaaactactaacccggtagcaacggagtcctatggacaagtggccacaaaccaccagagtgcccaagcacaggcgcagaccggctgggttcaaaaccaaggaatacttccgggtatggtttggcaggacagagatgtgtacctgcaaggacccatttgggccaaaattcctcacacggacggcaactttcacccttctccgctgatgggagggtttggaatgaagcacccgcctcctcagatcctcatcaaaaacacacctgtacctgcggatcctccaacggccttcaacaaggacaagctgaactctttcatcacccagtattctactggccaagtcagcgtggagatcgagtgggagctgcagaaggaaaacagcaagc

SEQ ID NO: 39 - protein, 250 aa, Unknown
  AAV-ScFv
DIVLTQSPASLAVSLGQRATISCRASQSVSSSTYNFIHWYQQKSGQPPKLLIKYASNLESGVPVRFSGSGSGTDFSLNIHPVEEEDTATYYCQHSWEIPYTFGGGAKLEIKGSTSGGGSGGGSGGGGSSQVQLKESGPGLVAPSQSLSITCTVSGFSLSGYGISWVRQPPGKRLEWLGLIWGDGTTDYNSALKSRLSISKDNSKSQVFLKMNSLQTDDTARYFCTRGPPAFYKYLYFDYWGQGTTLTVSS